European Patent Specification EP 3 554 485 B9, published September 27, 2023. Title: TREATMENT OF A DISEASE OF THE GASTROINTESTINAL TRACT WITH A JAK INHIBITOR. Applicant: Progenity Inc. The sequence listing filed with the application follows.

SEQUENCE LISTING (15 sequences)

SEQ ID NO: 1 - DNA, 5118 bp, Homo sapiens
ggggcgggacgggaggcggtgcgtcgctgagcgcaggccgcggcggccgcggagtatcctggagctgcagacagtgcgggcctgcgcccagtcccggctgtcctcgccgcgacccctcctcagccctgggcgcgcgcacgctggggccccgcggggctggccgcctagcgagcctgccggtcgaccccagccagcgcagcgacggggcgctgcctggcccaggcgcacacggaagtgcgcttctctgaagtagctttggaaagtagagaagaaaatccagtttgcttcttggagaacactggacagctgaataaatgcagtatctaaatataaaagaggactgcaatgccatggctttctgtgctaaaatgaggagctccaagaagactgaggtgaacctggaggcccctgagccaggggtggaagtgatcttctatctgtcggacagggagcccctccggctgggcagtggagagtacacagcagaggaactgtgcatcagggctgcacaggcatgccgtatctctcctctttgtcacaacctctttgccctgtatgacgagaacaccaagctctggtatgctccaaatcgcaccatcaccgttgatgacaagatgtccctccggctccactaccggatgaggttctatttcaccaattggcatggaaccaacgacaatgagcagtcagtgtggcgtcattctccaaagaagcagaaaaatggctacgagaaaaaaaagattccagatgcaacccctctccttgatgccagctcactggagtatctgtttgctcagggacagtatgatttggtgaaatgcctggctcctattcgagaccccaagaccgagcaggatggacatgatattgagaacgagtgtctagggatggctgtcctggccatctcacactatgccatgatgaagaagatgcagttgccagaactgcccaaggacatcagctacaagcgatatattccagaaacattgaataagtccatcagacagaggaaccttctcaccaggatgcggataaataatgttttcaaggatttcctaaaggaatttaacaacaagaccatttgtgacagcagcgtgtccacgcatgacctgaaggtgaaatacttggctaccttggaaactttgacaaaacattacggtgctgaaatatttgagacttccatgttactgatttcatcagaaaatgagatgaattggtttcattcgaatgacggtggaaacgttctctactacgaagtgatggtgactgggaatcttggaatccagtggaggcataaaccaaatgttgtttctgttgaaaaggaaaaaaataaactgaagcggaaaaaactggaaaataaacacaagaaggatgaggagaaaaacaagatccgggaagagtggaacaatttttcttacttccctgaaatcactcacattgtaataaaggagtctgtggtcagcattaacaagcaggacaacaagaaaatggaactgaagctctcttcccacgaggaggccttgtcctttgtgtccctggtagatggctacttccggctcacagcagatgcccatcattacctctgcaccgacgtggcccccccgttgatcgtccacaacatacagaatggctgtcatggtccaatctgtacagaatacgccatcaataaattgcggcaagaaggaagcgaggaggggatgtacgtgctgaggtggagctgcaccgactttgacaacatcctcatgaccgtcacctgctttgagaagtctgagcaggtgcagggtgcccagaagcagttcaagaactttcagatcgaggtgcagaagggccgctacagtctgcacggttcggaccgcagcttccccagcttgggagacctcatgagccacctcaagaagcagatcctgcgcacggataacatcagcttcatgctaaaacgctgctgccagcccaagccccgagaaatctccaacctgctggtggctactaagaaagcccaggagtggcagcccgtctaccccatgagccagctgagtttcgatcggatcctcaagaaggatctggtgcagggcgagcaccttgggagaggcacgagaacacacatctattctgggaccctgatggattacaaggatgacgaaggaacttctgaagagaagaagataaaagtgatcctcaaagtcttagaccccagccacagggatatttccctggccttcttcgaggcagccagcatgatgagacaggtctcccacaaacacatcgtgtacctctatggcgtctgtgtccgcgacgtggagaatatcatggtggaagagtttgtggaagggggtcctctggatctcttcatgcaccggaaaagcgatgtccttaccacaccatggaaattcaaagttgccaaacagctggccagtgccctgagctacttggaggataaagacctggtccatggaaatgtgtgtactaaaaacctcctcctggcccgtgagggcatcgacagtgagtgtggcccattcatcaagctcagtgaccccggcatccccattacggtgctgtctaggcaagaatgcattgaacgaatcccatggattgctcctgagtgtgttgaggactccaagaacctgagtgtggctgctgacaagtggagctttggaaccacgctctgggaaatctgctacaatggcgagatccccttgaaagacaagacgctgattgagaaagagagattctatgaaagccggtgcaggccagtgacaccatcatgtaaggagctggctgacctcatgacccgctgcatgaactatgaccccaatcagaggcctttcttccgagccatcatgagagacattaataagcttgaagagcagaatccagatattgtttcagaaaaaaaaccagcaactgaagtggaccccacacattttgaaaagcgcttcctaaagaggatccgtgacttgggagagggccactttgggaaggttgagctctgcaggtatgaccccgaaggggacaatacaggggagcaggtggctgttaaatctctgaagcctgagagtggaggtaaccacatagctgatctgaaaaaggaaatcgagatcttaaggaacctctatcatgagaacattgtgaagtacaaaggaatctgcacagaagacggaggaaatggtattaagctcatcatggaatttctgccttcgggaagccttaaggaatatcttccaaagaataagaacaaaataaacctcaaacagcagctaaaatatgccgttcagatttgtaaggggatggactatttgggttctcggcaatacgttcaccgggacttggcagcaagaaatgtccttgttgagagtgaacaccaagtgaaaattggagacttcggtttaaccaaagcaattgaaaccgataaggagtattacaccgtcaaggatgaccgggacagccctgtgttttggtatgctccagaatgtttaatgcaatctaaattttatattgcctctgacgtctggtcttttggagtcactctgcatgagctgctgacttactgtgattcagattctagtcccatggctttgttcctgaaaatgataggcccaacccatggccagatgacagtcacaagacttgtgaatacgttaaaagaaggaaaacgcctgccgtgcccacctaactgtccagatgaggtttatcaacttatgaggaaatgctgggaattccaaccatccaatcggacaagctttcagaaccttattgaaggatttgaagcacttttaaaataagaagcatgaataacatttaaattccacagattatcaagtccttctcctgcaacaaatgcccaagtcattttttaaaaatttctaatgaaagaagtttgtgttctgtccaaaaagtcactgaactcatacttcagtacatatacatgtataaggcacactgtagtgcttaatatgtgtaaggacttcctctttaaatttggtaccagtaacttagtgacacataatgacaaccaaaatatttgaaagcacttaagcactcctccttgtggaaagaatataccaccatttcatctggctagttcaccatcacaactgcattaccaaaaggggatttttgaaaacgaggagttgaccaaaataatatctgaagatgattgcttttccctgctgccagctgatctgaaatgttttgctggcacattaatcatagataaagaaagattgatggacttagccctcaaatttcagtatctatacagtactagaccatgcattcttaaaatattagataccaggtagtatatattgtttctgtacaaaaatgactgtattctctcaccagtaggacttaaactttgtttctccagtggcttagctcctgttcctttgggtgatcactagcacccatttttgagaaagctggttctacatggggggatagctgtggaatagataatttgctgcatgttaattctcaagaactaagcctgtgccagtgctttcctaagcagtatacctttaatcagaactcattcccagaacctggatgctattacacatgcttttaagaaacgtcaatgtatatccttttataactctaccactttggggcaagctattccagcactggttttgaatgctgtatgcaaccagtctgaataccacatacgctgcactgttcttagagggtttccatacttaccaccgatctacaagggttgatccctgtttttaccatcaatcatcaccctgtggtgcaacacttgaaagacccggctagaggcactatggacttcaggatccactagacagttttcagtttgcttggaggtagctgggtaatcaaaaatgtttagtcattgattcaatgtgaacgattacggtctttatgaccaagagtctgaaaatctttttgttatgctgtttagtattcgtttgatattgttacttttcacctgttgagcccaaattcaggattggttcagtggcagcaatgaagttgccatttaaatttgttcatagcctacatcaccaaggtctctgtgtcaaacctgtggccactctatatgcactttgtttactctttatacaaataaatatactaaagactttacatgca

SEQ ID NO: 2 - DNA, 5021 bp, Homo sapiens
agaagcggagcgtatacggaggaggcgggatgcatttctgcatcgagcgcacaaagttatctaaaacagttcatgctgctgaaaacctccttcctggcagatgtccctcaaccctactggtgcctggcttctgagacacacgcttctctgaagtagctttggaaagtagagaagaaaatccagtttgcttcttggagaacactggacagctgaataaatgcagtatctaaatataaaagaggactgcaatgccatggctttctgtgctaaaatgaggagctccaagaagactgaggtgaacctggaggcccctgagccaggggtggaagtgatcttctatctgtcggacagggagcccctccggctgggcagtggagagtacacagcagaggaactgtgcatcagggctgcacaggcatgccgtatctctcctctttgtcacaacctctttgccctgtatgacgagaacaccaagctctggtatgctccaaatcgcaccatcaccgttgatgacaagatgtccctccggctccactaccggatgaggttctatttcaccaattggcatggaaccaacgacaatgagcagtcagtgtggcgtcattctccaaagaagcagaaaaatggctacgagaaaaaaaagattccagatgcaacccctctccttgatgccagctcactggagtatctgtttgctcagggacagtatgatttggtgaaatgcctggctcctattcgagaccccaagaccgagcaggatggacatgatattgagaacgagtgtctagggatggctgtcctggccatctcacactatgccatgatgaagaagatgcagttgccagaactgcccaaggacatcagctacaagcgatatattccagaaacattgaataagtccatcagacagaggaaccttctcaccaggatgcggataaataatgttttcaaggatttcctaaaggaatttaacaacaagaccatttgtgacagcagcgtgtccacgcatgacctgaaggtgaaatacttggctaccttggaaactttgacaaaacattacggtgctgaaatatttgagacttccatgttactgatttcatcagaaaatgagatgaattggtttcattcgaatgacggtggaaacgttctctactacgaagtgatggtgactgggaatcttggaatccagtggaggcataaaccaaatgttgtttctgttgaaaaggaaaaaaataaactgaagcggaaaaaactggaaaataaacacaagaaggatgaggagaaaaacaagatccgggaagagtggaacaatttttcttacttccctgaaatcactcacattgtaataaaggagtctgtggtcagcattaacaagcaggacaacaagaaaatggaactgaagctctcttcccacgaggaggccttgtcctttgtgtccctggtagatggctacttccggctcacagcagatgcccatcattacctctgcaccgacgtggcccccccgttgatcgtccacaacatacagaatggctgtcatggtccaatctgtacagaatacgccatcaataaattgcggcaagaaggaagcgaggaggggatgtacgtgctgaggtggagctgcaccgactttgacaacatcctcatgaccgtcacctgctttgagaagtctgagcaggtgcagggtgcccagaagcagttcaagaactttcagatcgaggtgcagaagggccgctacagtctgcacggttcggaccgcagcttccccagcttgggagacctcatgagccacctcaagaagcagatcctgcgcacggataacatcagcttcatgctaaaacgctgctgccagcccaagccccgagaaatctccaacctgctggtggctactaagaaagcccaggagtggcagcccgtctaccccatgagccagctgagtttcgatcggatcctcaagaaggatctggtgcagggcgagcaccttgggagaggcacgagaacacacatctattctgggaccctgatggattacaaggatgacgaaggaacttctgaagagaagaagataaaagtgatcctcaaagtcttagaccccagccacagggatatttccctggccttcttcgaggcagccagcatgatgagacaggtctcccacaaacacatcgtgtacctctatggcgtctgtgtccgcgacgtggagaatatcatggtggaagagtttgtggaagggggtcctctggatctcttcatgcaccggaaaagcgatgtccttaccacaccatggaaattcaaagttgccaaacagctggccagtgccctgagctacttggaggataaagacctggtccatggaaatgtgtgtactaaaaacctcctcctggcccgtgagggcatcgacagtgagtgtggcccattcatcaagctcagtgaccccggcatccccattacggtgctgtctaggcaagaatgcattgaacgaatcccatggattgctcctgagtgtgttgaggactccaagaacctgagtgtggctgctgacaagtggagctttggaaccacgctctgggaaatctgctacaatggcgagatccccttgaaagacaagacgctgattgagaaagagagattctatgaaagccggtgcaggccagtgacaccatcatgtaaggagctggctgacctcatgacccgctgcatgaactatgaccccaatcagaggcctttcttccgagccatcatgagagacattaataagcttgaagagcagaatccagatattgtttcagaaaaaaaaccagcaactgaagtggaccccacacattttgaaaagcgcttcctaaagaggatccgtgacttgggagagggccactttgggaaggttgagctctgcaggtatgaccccgaaggggacaatacaggggagcaggtggctgttaaatctctgaagcctgagagtggaggtaaccacatagctgatctgaaaaaggaaatcgagatcttaaggaacctctatcatgagaacattgtgaagtacaaaggaatctgcacagaagacggaggaaatggtattaagctcatcatggaatttctgccttcgggaagccttaaggaatatcttccaaagaataagaacaaaataaacctcaaacagcagctaaaatatgccgttcagatttgtaaggggatggactatttgggttctcggcaatacgttcaccgggacttggcagcaagaaatgtccttgttgagagtgaacaccaagtgaaaattggagacttcggtttaaccaaagcaattgaaaccgataaggagtattacaccgtcaaggatgaccgggacagccctgtgttttggtatgctccagaatgtttaatgcaatctaaattttatattgcctctgacgtctggtcttttggagtcactctgcatgagctgctgacttactgtgattcagattctagtcccatggctttgttcctgaaaatgataggcccaacccatggccagatgacagtcacaagacttgtgaatacgttaaaagaaggaaaacgcctgccgtgcccacctaactgtccagatgaggtttatcaacttatgaggaaatgctgggaattccaaccatccaatcggacaagctttcagaaccttattgaaggatttgaagcacttttaaaataagaagcatgaataacatttaaattccacagattatcaagtccttctcctgcaacaaatgcccaagtcattttttaaaaatttctaatgaaagaagtttgtgttctgtccaaaaagtcactgaactcatacttcagtacatatacatgtataaggcacactgtagtgcttaatatgtgtaaggacttcctctttaaatttggtaccagtaacttagtgacacataatgacaaccaaaatatttgaaagcacttaagcactcctccttgtggaaagaatataccaccatttcatctggctagttcaccatcacaactgcattaccaaaaggggatttttgaaaacgaggagttgaccaaaataatatctgaagatgattgcttttccctgctgccagctgatctgaaatgttttgctggcacattaatcatagataaagaaagattgatggacttagccctcaaatttcagtatctatacagtactagaccatgcattcttaaaatattagataccaggtagtatatattgtttctgtacaaaaatgactgtattctctcaccagtaggacttaaactttgtttctccagtggcttagctcctgttcctttgggtgatcactagcacccatttttgagaaagctggttctacatggggggatagctgtggaatagataatttgctgcatgttaattctcaagaactaagcctgtgccagtgctttcctaagcagtatacctttaatcagaactcattcccagaacctggatgctattacacatgcttttaagaaacgtcaatgtatatccttttataactctaccactttggggcaagctattccagcactggttttgaatgctgtatgcaaccagtctgaataccacatacgctgcactgttcttagagggtttccatacttaccaccgatctacaagggttgatccctgtttttaccatcaatcatcaccctgtggtgcaacacttgaaagacccggctagaggcactatggacttcaggatccactagacagttttcagtttgcttggaggtagctgggtaatcaaaaatgtttagtcattgattcaatgtgaacgattacggtctttatgaccaagagtctgaaaatctttttgttatgctgtttagtattcgtttgatattgttacttttcacctgttgagcccaaattcaggattggttcagtggcagcaatgaagttgccatttaaatttgttcatagcctacatcaccaaggtctctgtgtcaaacctgtggccactctatatgcactttgtttactctttatacaaataaatatactaaagactttacatgca

SEQ ID NO: 3 - DNA, 5024 bp, Homo sapiens
atctatcacatggcagagatagaataaaaacagaaaaatggcgacggtcacgttgtggcgagccttgctgcgtcattagataatcctcatgcaaatagcgggaagaacaaaggaaggggagcccgggacccccgggggcgcagcgcttctctgaagtagctttggaaagtagagaagaaaatccagtttgcttcttggagaacactggacagctgaataaatgcagtatctaaatataaaagaggactgcaatgccatggctttctgtgctaaaatgaggagctccaagaagactgaggtgaacctggaggcccctgagccaggggtggaagtgatcttctatctgtcggacagggagcccctccggctgggcagtggagagtacacagcagaggaactgtgcatcagggctgcacaggcatgccgtatctctcctctttgtcacaacctctttgccctgtatgacgagaacaccaagctctggtatgctccaaatcgcaccatcaccgttgatgacaagatgtccctccggctccactaccggatgaggttctatttcaccaattggcatggaaccaacgacaatgagcagtcagtgtggcgtcattctccaaagaagcagaaaaatggctacgagaaaaaaaagattccagatgcaacccctctccttgatgccagctcactggagtatctgtttgctcagggacagtatgatttggtgaaatgcctggctcctattcgagaccccaagaccgagcaggatggacatgatattgagaacgagtgtctagggatggctgtcctggccatctcacactatgccatgatgaagaagatgcagttgccagaactgcccaaggacatcagctacaagcgatatattccagaaacattgaataagtccatcagacagaggaaccttctcaccaggatgcggataaataatgttttcaaggatttcctaaaggaatttaacaacaagaccatttgtgacagcagcgtgtccacgcatgacctgaaggtgaaatacttggctaccttggaaactttgacaaaacattacggtgctgaaatatttgagacttccatgttactgatttcatcagaaaatgagatgaattggtttcattcgaatgacggtggaaacgttctctactacgaagtgatggtgactgggaatcttggaatccagtggaggcataaaccaaatgttgtttctgttgaaaaggaaaaaaataaactgaagcggaaaaaactggaaaataaacacaagaaggatgaggagaaaaacaagatccgggaagagtggaacaatttttcttacttccctgaaatcactcacattgtaataaaggagtctgtggtcagcattaacaagcaggacaacaagaaaatggaactgaagctctcttcccacgaggaggccttgtcctttgtgtccctggtagatggctacttccggctcacagcagatgcccatcattacctctgcaccgacgtggcccccccgttgatcgtccacaacatacagaatggctgtcatggtccaatctgtacagaatacgccatcaataaattgcggcaagaaggaagcgaggaggggatgtacgtgctgaggtggagctgcaccgactttgacaacatcctcatgaccgtcacctgctttgagaagtctgagcaggtgcagggtgcccagaagcagttcaagaactttcagatcgaggtgcagaagggccgctacagtctgcacggttcggaccgcagcttccccagcttgggagacctcatgagccacctcaagaagcagatcctgcgcacggataacatcagcttcatgctaaaacgctgctgccagcccaagccccgagaaatctccaacctgctggtggctactaagaaagcccaggagtggcagcccgtctaccccatgagccagctgagtttcgatcggatcctcaagaaggatctggtgcagggcgagcaccttgggagaggcacgagaacacacatctattctgggaccctgatggattacaaggatgacgaaggaacttctgaagagaagaagataaaagtgatcctcaaagtcttagaccccagccacagggatatttccctggccttcttcgaggcagccagcatgatgagacaggtctcccacaaacacatcgtgtacctctatggcgtctgtgtccgcgacgtggagaatatcatggtggaagagtttgtggaagggggtcctctggatctcttcatgcaccggaaaagcgatgtccttaccacaccatggaaattcaaagttgccaaacagctggccagtgccctgagctacttggaggataaagacctggtccatggaaatgtgtgtactaaaaacctcctcctggcccgtgagggcatcgacagtgagtgtggcccattcatcaagctcagtgaccccggcatccccattacggtgctgtctaggcaagaatgcattgaacgaatcccatggattgctcctgagtgtgttgaggactccaagaacctgagtgtggctgctgacaagtggagctttggaaccacgctctgggaaatctgctacaatggcgagatccccttgaaagacaagacgctgattgagaaagagagattctatgaaagccggtgcaggccagtgacaccatcatgtaaggagctggctgacctcatgacccgctgcatgaactatgaccccaatcagaggcctttcttccgagccatcatgagagacattaataagcttgaagagcagaatccagatattgtttcagaaaaaaaaccagcaactgaagtggaccccacacattttgaaaagcgcttcctaaagaggatccgtgacttgggagagggccactttgggaaggttgagctctgcaggtatgaccccgaaggggacaatacaggggagcaggtggctgttaaatctctgaagcctgagagtggaggtaaccacatagctgatctgaaaaaggaaatcgagatcttaaggaacctctatcatgagaacattgtgaagtacaaaggaatctgcacagaagacggaggaaatggtattaagctcatcatggaatttctgccttcgggaagccttaaggaatatcttccaaagaataagaacaaaataaacctcaaacagcagctaaaatatgccgttcagatttgtaaggggatggactatttgggttctcggcaatacgttcaccgggacttggcagcaagaaatgtccttgttgagagtgaacaccaagtgaaaattggagacttcggtttaaccaaagcaattgaaaccgataaggagtattacaccgtcaaggatgaccgggacagccctgtgttttggtatgctccagaatgtttaatgcaatctaaattttatattgcctctgacgtctggtcttttggagtcactctgcatgagctgctgacttactgtgattcagattctagtcccatggctttgttcctgaaaatgataggcccaacccatggccagatgacagtcacaagacttgtgaatacgttaaaagaaggaaaacgcctgccgtgcccacctaactgtccagatgaggtttatcaacttatgaggaaatgctgggaattccaaccatccaatcggacaagctttcagaaccttattgaaggatttgaagcacttttaaaataagaagcatgaataacatttaaattccacagattatcaagtccttctcctgcaacaaatgcccaagtcattttttaaaaatttctaatgaaagaagtttgtgttctgtccaaaaagtcactgaactcatacttcagtacatatacatgtataaggcacactgtagtgcttaatatgtgtaaggacttcctctttaaatttggtaccagtaacttagtgacacataatgacaaccaaaatatttgaaagcacttaagcactcctccttgtggaaagaatataccaccatttcatctggctagttcaccatcacaactgcattaccaaaaggggatttttgaaaacgaggagttgaccaaaataatatctgaagatgattgcttttccctgctgccagctgatctgaaatgttttgctggcacattaatcatagataaagaaagattgatggacttagccctcaaatttcagtatctatacagtactagaccatgcattcttaaaatattagataccaggtagtatatattgtttctgtacaaaaatgactgtattctctcaccagtaggacttaaactttgtttctccagtggcttagctcctgttcctttgggtgatcactagcacccatttttgagaaagctggttctacatggggggatagctgtggaatagataatttgctgcatgttaattctcaagaactaagcctgtgccagtgctttcctaagcagtatacctttaatcagaactcattcccagaacctggatgctattacacatgcttttaagaaacgtcaatgtatatccttttataactctaccactttggggcaagctattccagcactggttttgaatgctgtatgcaaccagtctgaataccacatacgctgcactgttcttagagggtttccatacttaccaccgatctacaagggttgatccctgtttttaccatcaatcatcaccctgtggtgcaacacttgaaagacccggctagaggcactatggacttcaggatccactagacagttttcagtttgcttggaggtagctgggtaatcaaaaatgtttagtcattgattcaatgtgaacgattacggtctttatgaccaagagtctgaaaatctttttgttatgctgtttagtattcgtttgatattgttacttttcacctgttgagcccaaattcaggattggttcagtggcagcaatgaagttgccatttaaatttgttcatagcctacatcaccaaggtctctgtgtcaaacctgtggccactctatatgcactttgtttactctttatacaaataaatatactaaagactttacatgca

SEQ ID NO: 4 - DNA, 5283 bp, Homo sapiens
atctatcacatggcagagatagaataaaaacagaaaaatggcgacggtcacgttgtggcgagccttgctgcgtcattagataatcctcatgcaaatagcgggaagaacaaaggaaggggagcccgggacccccgggggcgcaggatccggcgggaggagtctaagaggaggaggcggcggtgccggaggaggaggaggagggagggagaagagaggaagaccggagtccccgcggcggcggcggtccggagagagggcgagccccgcgcggcgccggggaccgggcgctaccacgaggccgggacgctggagtctgggttatctaaaacagttcatgctgctgaaaacctccttcctggcagatgtccctcaaccctactggtgcctggcttctgagacacacgcttctctgaagtagctttggaaagtagagaagaaaatccagtttgcttcttggagaacactggacagctgaataaatgcagtatctaaatataaaagaggactgcaatgccatggctttctgtgctaaaatgaggagctccaagaagactgaggtgaacctggaggcccctgagccaggggtggaagtgatcttctatctgtcggacagggagcccctccggctgggcagtggagagtacacagcagaggaactgtgcatcagggctgcacaggcatgccgtatctctcctctttgtcacaacctctttgccctgtatgacgagaacaccaagctctggtatgctccaaatcgcaccatcaccgttgatgacaagatgtccctccggctccactaccggatgaggttctatttcaccaattggcatggaaccaacgacaatgagcagtcagtgtggcgtcattctccaaagaagcagaaaaatggctacgagaaaaaaaagattccagatgcaacccctctccttgatgccagctcactggagtatctgtttgctcagggacagtatgatttggtgaaatgcctggctcctattcgagaccccaagaccgagcaggatggacatgatattgagaacgagtgtctagggatggctgtcctggccatctcacactatgccatgatgaagaagatgcagttgccagaactgcccaaggacatcagctacaagcgatatattccagaaacattgaataagtccatcagacagaggaaccttctcaccaggatgcggataaataatgttttcaaggatttcctaaaggaatttaacaacaagaccatttgtgacagcagcgtgtccacgcatgacctgaaggtgaaatacttggctaccttggaaactttgacaaaacattacggtgctgaaatatttgagacttccatgttactgatttcatcagaaaatgagatgaattggtttcattcgaatgacggtggaaacgttctctactacgaagtgatggtgactgggaatcttggaatccagtggaggcataaaccaaatgttgtttctgttgaaaaggaaaaaaataaactgaagcggaaaaaactggaaaataaacacaagaaggatgaggagaaaaacaagatccgggaagagtggaacaatttttcttacttccctgaaatcactcacattgtaataaaggagtctgtggtcagcattaacaagcaggacaacaagaaaatggaactgaagctctcttcccacgaggaggccttgtcctttgtgtccctggtagatggctacttccggctcacagcagatgcccatcattacctctgcaccgacgtggcccccccgttgatcgtccacaacatacagaatggctgtcatggtccaatctgtacagaatacgccatcaataaattgcggcaagaaggaagcgaggaggggatgtacgtgctgaggtggagctgcaccgactttgacaacatcctcatgaccgtcacctgctttgagaagtctgagcaggtgcagggtgcccagaagcagttcaagaactttcagatcgaggtgcagaagggccgctacagtctgcacggttcggaccgcagcttccccagcttgggagacctcatgagccacctcaagaagcagatcctgcgcacggataacatcagcttcatgctaaaacgctgctgccagcccaagccccgagaaatctccaacctgctggtggctactaagaaagcccaggagtggcagcccgtctaccccatgagccagctgagtttcgatcggatcctcaagaaggatctggtgcagggcgagcaccttgggagaggcacgagaacacacatctattctgggaccctgatggattacaaggatgacgaaggaacttctgaagagaagaagataaaagtgatcctcaaagtcttagaccccagccacagggatatttccctggccttcttcgaggcagccagcatgatgagacaggtctcccacaaacacatcgtgtacctctatggcgtctgtgtccgcgacgtggagaatatcatggtggaagagtttgtggaagggggtcctctggatctcttcatgcaccggaaaagcgatgtccttaccacaccatggaaattcaaagttgccaaacagctggccagtgccctgagctacttggaggataaagacctggtccatggaaatgtgtgtactaaaaacctcctcctggcccgtgagggcatcgacagtgagtgtggcccattcatcaagctcagtgaccccggcatccccattacggtgctgtctaggcaagaatgcattgaacgaatcccatggattgctcctgagtgtgttgaggactccaagaacctgagtgtggctgctgacaagtggagctttggaaccacgctctgggaaatctgctacaatggcgagatccccttgaaagacaagacgctgattgagaaagagagattctatgaaagccggtgcaggccagtgacaccatcatgtaaggagctggctgacctcatgacccgctgcatgaactatgaccccaatcagaggcctttcttccgagccatcatgagagacattaataagcttgaagagcagaatccagatattgtttcagaaaaaaaaccagcaactgaagtggaccccacacattttgaaaagcgcttcctaaagaggatccgtgacttgggagagggccactttgggaaggttgagctctgcaggtatgaccccgaaggggacaatacaggggagcaggtggctgttaaatctctgaagcctgagagtggaggtaaccacatagctgatctgaaaaaggaaatcgagatcttaaggaacctctatcatgagaacattgtgaagtacaaaggaatctgcacagaagacggaggaaatggtattaagctcatcatggaatttctgccttcgggaagccttaaggaatatcttccaaagaataagaacaaaataaacctcaaacagcagctaaaatatgccgttcagatttgtaaggggatggactatttgggttctcggcaatacgttcaccgggacttggcagcaagaaatgtccttgttgagagtgaacaccaagtgaaaattggagacttcggtttaaccaaagcaattgaaaccgataaggagtattacaccgtcaaggatgaccgggacagccctgtgttttggtatgctccagaatgtttaatgcaatctaaattttatattgcctctgacgtctggtcttttggagtcactctgcatgagctgctgacttactgtgattcagattctagtcccatggctttgttcctgaaaatgataggcccaacccatggccagatgacagtcacaagacttgtgaatacgttaaaagaaggaaaacgcctgccgtgcccacctaactgtccagatgaggtttatcaacttatgaggaaatgctgggaattccaaccatccaatcggacaagctttcagaaccttattgaaggatttgaagcacttttaaaataagaagcatgaataacatttaaattccacagattatcaagtccttctcctgcaacaaatgcccaagtcattttttaaaaatttctaatgaaagaagtttgtgttctgtccaaaaagtcactgaactcatacttcagtacatatacatgtataaggcacactgtagtgcttaatatgtgtaaggacttcctctttaaatttggtaccagtaacttagtgacacataatgacaaccaaaatatttgaaagcacttaagcactcctccttgtggaaagaatataccaccatttcatctggctagttcaccatcacaactgcattaccaaaaggggatttttgaaaacgaggagttgaccaaaataatatctgaagatgattgcttttccctgctgccagctgatctgaaatgttttgctggcacattaatcatagataaagaaagattgatggacttagccctcaaatttcagtatctatacagtactagaccatgcattcttaaaatattagataccaggtagtatatattgtttctgtacaaaaatgactgtattctctcaccagtaggacttaaactttgtttctccagtggcttagctcctgttcctttgggtgatcactagcacccatttttgagaaagctggttctacatggggggatagctgtggaatagataatttgctgcatgttaattctcaagaactaagcctgtgccagtgctttcctaagcagtatacctttaatcagaactcattcccagaacctggatgctattacacatgcttttaagaaacgtcaatgtatatccttttataactctaccactttggggcaagctattccagcactggttttgaatgctgtatgcaaccagtctgaataccacatacgctgcactgttcttagagggtttccatacttaccaccgatctacaagggttgatccctgtttttaccatcaatcatcaccctgtggtgcaacacttgaaagacccggctagaggcactatggacttcaggatccactagacagttttcagtttgcttggaggtagctgggtaatcaaaaatgtttagtcattgattcaatgtgaacgattacggtctttatgaccaagagtctgaaaatctttttgttatgctgtttagtattcgtttgatattgttacttttcacctgttgagcccaaattcaggattggttcagtggcagcaatgaagttgccatttaaatttgttcatagcctacatcaccaaggtctctgtgtcaaacctgtggccactctatatgcactttgtttactctttatacaaataaatatactaaagactttacatgca

SEQ ID NO: 5 - DNA, 5199 bp, Homo sapiens
atctatcacatggcagagatagaataaaaacagaaaaatggcgacggtcacgttgtggcgagccttgctgcgtcattagataatcctcatgcaaatagcgggaagaacaaaggaaggggagcccgggacccccgggggcgcaggatccggcgggaggagtctaagaggaggaggcggcggtgccggaggaggaggaggagggagggagaagagaggaagaccggagtccccgcggcggcggcggtccggagagagggcgagccccgcgcggcgccggggaccgggcgctaccacgaggccgggacgctggagtctgggcgcttctctgaagtagctttggaaagtagagaagaaaatccagtttgcttcttggagaacactggacagctgaataaatgcagtatctaaatataaaagaggactgcaatgccatggctttctgtgctaaaatgaggagctccaagaagactgaggtgaacctggaggcccctgagccaggggtggaagtgatcttctatctgtcggacagggagcccctccggctgggcagtggagagtacacagcagaggaactgtgcatcagggctgcacaggcatgccgtatctctcctctttgtcacaacctctttgccctgtatgacgagaacaccaagctctggtatgctccaaatcgcaccatcaccgttgatgacaagatgtccctccggctccactaccggatgaggttctatttcaccaattggcatggaaccaacgacaatgagcagtcagtgtggcgtcattctccaaagaagcagaaaaatggctacgagaaaaaaaagattccagatgcaacccctctccttgatgccagctcactggagtatctgtttgctcagggacagtatgatttggtgaaatgcctggctcctattcgagaccccaagaccgagcaggatggacatgatattgagaacgagtgtctagggatggctgtcctggccatctcacactatgccatgatgaagaagatgcagttgccagaactgcccaaggacatcagctacaagcgatatattccagaaacattgaataagtccatcagacagaggaaccttctcaccaggatgcggataaataatgttttcaaggatttcctaaaggaatttaacaacaagaccatttgtgacagcagcgtgtccacgcatgacctgaaggtgaaatacttggctaccttggaaactttgacaaaacattacggtgctgaaatatttgagacttccatgttactgatttcatcagaaaatgagatgaattggtttcattcgaatgacggtggaaacgttctctactacgaagtgatggtgactgggaatcttggaatccagtggaggcataaaccaaatgttgtttctgttgaaaaggaaaaaaataaactgaagcggaaaaaactggaaaataaacacaagaaggatgaggagaaaaacaagatccgggaagagtggaacaatttttcttacttccctgaaatcactcacattgtaataaaggagtctgtggtcagcattaacaagcaggacaacaagaaaatggaactgaagctctcttcccacgaggaggccttgtcctttgtgtccctggtagatggctacttccggctcacagcagatgcccatcattacctctgcaccgacgtggcccccccgttgatcgtccacaacatacagaatggctgtcatggtccaatctgtacagaatacgccatcaataaattgcggcaagaaggaagcgaggaggggatgtacgtgctgaggtggagctgcaccgactttgacaacatcctcatgaccgtcacctgctttgagaagtctgagcaggtgcagggtgcccagaagcagttcaagaactttcagatcgaggtgcagaagggccgctacagtctgcacggttcggaccgcagcttccccagcttgggagacctcatgagccacctcaagaagcagatcctgcgcacggataacatcagcttcatgctaaaacgctgctgccagcccaagccccgagaaatctccaacctgctggtggctactaagaaagcccaggagtggcagcccgtctaccccatgagccagctgagtttcgatcggatcctcaagaaggatctggtgcagggcgagcaccttgggagaggcacgagaacacacatctattctgggaccctgatggattacaaggatgacgaaggaacttctgaagagaagaagataaaagtgatcctcaaagtcttagaccccagccacagggatatttccctggccttcttcgaggcagccagcatgatgagacaggtctcccacaaacacatcgtgtacctctatggcgtctgtgtccgcgacgtggagaatatcatggtggaagagtttgtggaagggggtcctctggatctcttcatgcaccggaaaagcgatgtccttaccacaccatggaaattcaaagttgccaaacagctggccagtgccctgagctacttggaggataaagacctggtccatggaaatgtgtgtactaaaaacctcctcctggcccgtgagggcatcgacagtgagtgtggcccattcatcaagctcagtgaccccggcatccccattacggtgctgtctaggcaagaatgcattgaacgaatcccatggattgctcctgagtgtgttgaggactccaagaacctgagtgtggctgctgacaagtggagctttggaaccacgctctgggaaatctgctacaatggcgagatccccttgaaagacaagacgctgattgagaaagagagattctatgaaagccggtgcaggccagtgacaccatcatgtaaggagctggctgacctcatgacccgctgcatgaactatgaccccaatcagaggcctttcttccgagccatcatgagagacattaataagcttgaagagcagaatccagatattgtttcagaaaaaaaaccagcaactgaagtggaccccacacattttgaaaagcgcttcctaaagaggatccgtgacttgggagagggccactttgggaaggttgagctctgcaggtatgaccccgaaggggacaatacaggggagcaggtggctgttaaatctctgaagcctgagagtggaggtaaccacatagctgatctgaaaaaggaaatcgagatcttaaggaacctctatcatgagaacattgtgaagtacaaaggaatctgcacagaagacggaggaaatggtattaagctcatcatggaatttctgccttcgggaagccttaaggaatatcttccaaagaataagaacaaaataaacctcaaacagcagctaaaatatgccgttcagatttgtaaggggatggactatttgggttctcggcaatacgttcaccgggacttggcagcaagaaatgtccttgttgagagtgaacaccaagtgaaaattggagacttcggtttaaccaaagcaattgaaaccgataaggagtattacaccgtcaaggatgaccgggacagccctgtgttttggtatgctccagaatgtttaatgcaatctaaattttatattgcctctgacgtctggtcttttggagtcactctgcatgagctgctgacttactgtgattcagattctagtcccatggctttgttcctgaaaatgataggcccaacccatggccagatgacagtcacaagacttgtgaatacgttaaaagaaggaaaacgcctgccgtgcccacctaactgtccagatgaggtttatcaacttatgaggaaatgctgggaattccaaccatccaatcggacaagctttcagaaccttattgaaggatttgaagcacttttaaaataagaagcatgaataacatttaaattccacagattatcaagtccttctcctgcaacaaatgcccaagtcattttttaaaaatttctaatgaaagaagtttgtgttctgtccaaaaagtcactgaactcatacttcagtacatatacatgtataaggcacactgtagtgcttaatatgtgtaaggacttcctctttaaatttggtaccagtaacttagtgacacataatgacaaccaaaatatttgaaagcacttaagcactcctccttgtggaaagaatataccaccatttcatctggctagttcaccatcacaactgcattaccaaaaggggatttttgaaaacgaggagttgaccaaaataatatctgaagatgattgcttttccctgctgccagctgatctgaaatgttttgctggcacattaatcatagataaagaaagattgatggacttagccctcaaatttcagtatctatacagtactagaccatgcattcttaaaatattagataccaggtagtatatattgtttctgtacaaaaatgactgtattctctcaccagtaggacttaaactttgtttctccagtggcttagctcctgttcctttgggtgatcactagcacccatttttgagaaagctggttctacatggggggatagctgtggaatagataatttgctgcatgttaattctcaagaactaagcctgtgccagtgctttcctaagcagtatacctttaatcagaactcattcccagaacctggatgctattacacatgcttttaagaaacgtcaatgtatatccttttataactctaccactttggggcaagctattccagcactggttttgaatgctgtatgcaaccagtctgaataccacatacgctgcactgttcttagagggtttccatacttaccaccgatctacaagggttgatccctgtttttaccatcaatcatcaccctgtggtgcaacacttgaaagacccggctagaggcactatggacttcaggatccactagacagttttcagtttgcttggaggtagctgggtaatcaaaaatgtttagtcattgattcaatgtgaacgattacggtctttatgaccaagagtctgaaaatctttttgttatgctgtttagtattcgtttgatattgttacttttcacctgttgagcccaaattcaggattggttcagtggcagcaatgaagttgccatttaaatttgttcatagcctacatcaccaaggtctctgtgtcaaacctgtggccactctatatgcactttgtttactctttatacaaataaatatactaaagactttacatgca

SEQ ID NO: 6 - DNA, 5202 bp, Homo sapiens
ggggcgggacgggaggcggtgcgtcgctgagcgcaggccgcggcggccgcggagtatcctggagctgcagacagtgcgggcctgcgcccagtcccggctgtcctcgccgcgacccctcctcagccctgggcgcgcgcacgctggggccccgcggggctggccgcctagcgagcctgccggtcgaccccagccagcgcagcgacggggcgctgcctggcccaggcgcacacggaagtgttatctaaaacagttcatgctgctgaaaacctccttcctggcagatgtccctcaaccctactggtgcctggcttctgagacacacgcttctctgaagtagctttggaaagtagagaagaaaatccagtttgcttcttggagaacactggacagctgaataaatgcagtatctaaatataaaagaggactgcaatgccatggctttctgtgctaaaatgaggagctccaagaagactgaggtgaacctggaggcccctgagccaggggtggaagtgatcttctatctgtcggacagggagcccctccggctgggcagtggagagtacacagcagaggaactgtgcatcagggctgcacaggcatgccgtatctctcctctttgtcacaacctctttgccctgtatgacgagaacaccaagctctggtatgctccaaatcgcaccatcaccgttgatgacaagatgtccctccggctccactaccggatgaggttctatttcaccaattggcatggaaccaacgacaatgagcagtcagtgtggcgtcattctccaaagaagcagaaaaatggctacgagaaaaaaaagattccagatgcaacccctctccttgatgccagctcactggagtatctgtttgctcagggacagtatgatttggtgaaatgcctggctcctattcgagaccccaagaccgagcaggatggacatgatattgagaacgagtgtctagggatggctgtcctggccatctcacactatgccatgatgaagaagatgcagttgccagaactgcccaaggacatcagctacaagcgatatattccagaaacattgaataagtccatcagacagaggaaccttctcaccaggatgcggataaataatgttttcaaggatttcctaaaggaatttaacaacaagaccatttgtgacagcagcgtgtccacgcatgacctgaaggtgaaatacttggctaccttggaaactttgacaaaacattacggtgctgaaatatttgagacttccatgttactgatttcatcagaaaatgagatgaattggtttcattcgaatgacggtggaaacgttctctactacgaagtgatggtgactgggaatcttggaatccagtggaggcataaaccaaatgttgtttctgttgaaaaggaaaaaaataaactgaagcggaaaaaactggaaaataaacacaagaaggatgaggagaaaaacaagatccgggaagagtggaacaatttttcttacttccctgaaatcactcacattgtaataaaggagtctgtggtcagcattaacaagcaggacaacaagaaaatggaactgaagctctcttcccacgaggaggccttgtcctttgtgtccctggtagatggctacttccggctcacagcagatgcccatcattacctctgcaccgacgtggcccccccgttgatcgtccacaacatacagaatggctgtcatggtccaatctgtacagaatacgccatcaataaattgcggcaagaaggaagcgaggaggggatgtacgtgctgaggtggagctgcaccgactttgacaacatcctcatgaccgtcacctgctttgagaagtctgagcaggtgcagggtgcccagaagcagttcaagaactttcagatcgaggtgcagaagggccgctacagtctgcacggttcggaccgcagcttccccagcttgggagacctcatgagccacctcaagaagcagatcctgcgcacggataacatcagcttcatgctaaaacgctgctgccagcccaagccccgagaaatctccaacctgctggtggctactaagaaagcccaggagtggcagcccgtctaccccatgagccagctgagtttcgatcggatcctcaagaaggatctggtgcagggcgagcaccttgggagaggcacgagaacacacatctattctgggaccctgatggattacaaggatgacgaaggaacttctgaagagaagaagataaaagtgatcctcaaagtcttagaccccagccacagggatatttccctggccttcttcgaggcagccagcatgatgagacaggtctcccacaaacacatcgtgtacctctatggcgtctgtgtccgcgacgtggagaatatcatggtggaagagtttgtggaagggggtcctctggatctcttcatgcaccggaaaagcgatgtccttaccacaccatggaaattcaaagttgccaaacagctggccagtgccctgagctacttggaggataaagacctggtccatggaaatgtgtgtactaaaaacctcctcctggcccgtgagggcatcgacagtgagtgtggcccattcatcaagctcagtgaccccggcatccccattacggtgctgtctaggcaagaatgcattgaacgaatcccatggattgctcctgagtgtgttgaggactccaagaacctgagtgtggctgctgacaagtggagctttggaaccacgctctgggaaatctgctacaatggcgagatccccttgaaagacaagacgctgattgagaaagagagattctatgaaagccggtgcaggccagtgacaccatcatgtaaggagctggctgacctcatgacccgctgcatgaactatgaccccaatcagaggcctttcttccgagccatcatgagagacattaataagcttgaagagcagaatccagatattgtttcagaaaaaaaaccagcaactgaagtggaccccacacattttgaaaagcgcttcctaaagaggatccgtgacttgggagagggccactttgggaaggttgagctctgcaggtatgaccccgaaggggacaatacaggggagcaggtggctgttaaatctctgaagcctgagagtggaggtaaccacatagctgatctgaaaaaggaaatcgagatcttaaggaacctctatcatgagaacattgtgaagtacaaaggaatctgcacagaagacggaggaaatggtattaagctcatcatggaatttctgccttcgggaagccttaaggaatatcttccaaagaataagaacaaaataaacctcaaacagcagctaaaatatgccgttcagatttgtaaggggatggactatttgggttctcggcaatacgttcaccgggacttggcagcaagaaatgtccttgttgagagtgaacaccaagtgaaaattggagacttcggtttaaccaaagcaattgaaaccgataaggagtattacaccgtcaaggatgaccgggacagccctgtgttttggtatgctccagaatgtttaatgcaatctaaattttatattgcctctgacgtctggtcttttggagtcactctgcatgagctgctgacttactgtgattcagattctagtcccatggctttgttcctgaaaatgataggcccaacccatggccagatgacagtcacaagacttgtgaatacgttaaaagaaggaaaacgcctgccgtgcccacctaactgtccagatgaggtttatcaacttatgaggaaatgctgggaattccaaccatccaatcggacaagctttcagaaccttattgaaggatttgaagcacttttaaaataagaagcatgaataacatttaaattccacagattatcaagtccttctcctgcaacaaatgcccaagtcattttttaaaaatttctaatgaaagaagtttgtgttctgtccaaaaagtcactgaactcatacttcagtacatatacatgtataaggcacactgtagtgcttaatatgtgtaaggacttcctctttaaatttggtaccagtaacttagtgacacataatgacaaccaaaatatttgaaagcacttaagcactcctccttgtggaaagaatataccaccatttcatctggctagttcaccatcacaactgcattaccaaaaggggatttttgaaaacgaggagttgaccaaaataatatctgaagatgattgcttttccctgctgccagctgatctgaaatgttttgctggcacattaatcatagataaagaaagattgatggacttagccctcaaatttcagtatctatacagtactagaccatgcattcttaaaatattagataccaggtagtatatattgtttctgtacaaaaatgactgtattctctcaccagtaggacttaaactttgtttctccagtggcttagctcctgttcctttgggtgatcactagcacccatttttgagaaagctggttctacatggggggatagctgtggaatagataatttgctgcatgttaattctcaagaactaagcctgtgccagtgctttcctaagcagtatacctttaatcagaactcattcccagaacctggatgctattacacatgcttttaagaaacgtcaatgtatatccttttataactctaccactttggggcaagctattccagcactggttttgaatgctgtatgcaaccagtctgaataccacatacgctgcactgttcttagagggtttccatacttaccaccgatctacaagggttgatccctgtttttaccatcaatcatcaccctgtggtgcaacacttgaaagacccggctagaggcactatggacttcaggatccactagacagttttcagtttgcttggaggtagctgggtaatcaaaaatgtttagtcattgattcaatgtgaacgattacggtctttatgaccaagagtctgaaaatctttttgttatgctgtttagtattcgtttgatattgttacttttcacctgttgagcccaaattcaggattggttcagtggcagcaatgaagttgccatttaaatttgttcatagcctacatcaccaaggtctctgtgtcaaacctgtggccactctatatgcactttgtttactctttatacaaataaatatactaaagactttacatgca

SEQ ID NO: 7 - DNA, 4937 bp, Homo sapiens
agaagcggagcgtatacggaggaggcgggatgcatttctgcatcgagcgcacaaagcgcttctctgaagtagctttggaaagtagagaagaaaatccagtttgcttcttggagaacactggacagctgaataaatgcagtatctaaatataaaagaggactgcaatgccatggctttctgtgctaaaatgaggagctccaagaagactgaggtgaacctggaggcccctgagccaggggtggaagtgatcttctatctgtcggacagggagcccctccggctgggcagtggagagtacacagcagaggaactgtgcatcagggctgcacaggcatgccgtatctctcctctttgtcacaacctctttgccctgtatgacgagaacaccaagctctggtatgctccaaatcgcaccatcaccgttgatgacaagatgtccctccggctccactaccggatgaggttctatttcaccaattggcatggaaccaacgacaatgagcagtcagtgtggcgtcattctccaaagaagcagaaaaatggctacgagaaaaaaaagattccagatgcaacccctctccttgatgccagctcactggagtatctgtttgctcagggacagtatgatttggtgaaatgcctggctcctattcgagaccccaagaccgagcaggatggacatgatattgagaacgagtgtctagggatggctgtcctggccatctcacactatgccatgatgaagaagatgcagttgccagaactgcccaaggacatcagctacaagcgatatattccagaaacattgaataagtccatcagacagaggaaccttctcaccaggatgcggataaataatgttttcaaggatttcctaaaggaatttaacaacaagaccatttgtgacagcagcgtgtccacgcatgacctgaaggtgaaatacttggctaccttggaaactttgacaaaacattacggtgctgaaatatttgagacttccatgttactgatttcatcagaaaatgagatgaattggtttcattcgaatgacggtggaaacgttctctactacgaagtgatggtgactgggaatcttggaatccagtggaggcataaaccaaatgttgtttctgttgaaaaggaaaaaaataaactgaagcggaaaaaactggaaaataaacacaagaaggatgaggagaaaaacaagatccgggaagagtggaacaatttttcttacttccctgaaatcactcacattgtaataaaggagtctgtggtcagcattaacaagcaggacaacaagaaaatggaactgaagctctcttcccacgaggaggccttgtcctttgtgtccctggtagatggctacttccggctcacagcagatgcccatcattacctctgcaccgacgtggcccccccgttgatcgtccacaacatacagaatggctgtcatggtccaatctgtacagaatacgccatcaataaattgcggcaagaaggaagcgaggaggggatgtacgtgctgaggtggagctgcaccgactttgacaacatcctcatgaccgtcacctgctttgagaagtctgagcaggtgcagggtgcccagaagcagttcaagaactttcagatcgaggtgcagaagggccgctacagtctgcacggttcggaccgcagcttccccagcttgggagacctcatgagccacctcaagaagcagatcctgcgcacggataacatcagcttcatgctaaaacgctgctgccagcccaagccccgagaaatctccaacctgctggtggctactaagaaagcccaggagtggcagcccgtctaccccatgagccagctgagtttcgatcggatcctcaagaaggatctggtgcagggcgagcaccttgggagaggcacgagaacacacatctattctgggaccctgatggattacaaggatgacgaaggaacttctgaagagaagaagataaaagtgatcctcaaagtcttagaccccagccacagggatatttccctggccttcttcgaggcagccagcatgatgagacaggtctcccacaaacacatcgtgtacctctatggcgtctgtgtccgcgacgtggagaatatcatggtggaagagtttgtggaagggggtcctctggatctcttcatgcaccggaaaagcgatgtccttaccacaccatggaaattcaaagttgccaaacagctggccagtgccctgagctacttggaggataaagacctggtccatggaaatgtgtgtactaaaaacctcctcctggcccgtgagggcatcgacagtgagtgtggcccattcatcaagctcagtgaccccggcatccccattacggtgctgtctaggcaagaatgcattgaacgaatcccatggattgctcctgagtgtgttgaggactccaagaacctgagtgtggctgctgacaagtggagctttggaaccacgctctgggaaatctgctacaatggcgagatccccttgaaagacaagacgctgattgagaaagagagattctatgaaagccggtgcaggccagtgacaccatcatgtaaggagctggctgacctcatgacccgctgcatgaactatgaccccaatcagaggcctttcttccgagccatcatgagagacattaataagcttgaagagcagaatccagatattgtttcagaaaaaaaaccagcaactgaagtggaccccacacattttgaaaagcgcttcctaaagaggatccgtgacttgggagagggccactttgggaaggttgagctctgcaggtatgaccccgaaggggacaatacaggggagcaggtggctgttaaatctctgaagcctgagagtggaggtaaccacatagctgatctgaaaaaggaaatcgagatcttaaggaacctctatcatgagaacattgtgaagtacaaaggaatctgcacagaagacggaggaaatggtattaagctcatcatggaatttctgccttcgggaagccttaaggaatatcttccaaagaataagaacaaaataaacctcaaacagcagctaaaatatgccgttcagatttgtaaggggatggactatttgggttctcggcaatacgttcaccgggacttggcagcaagaaatgtccttgttgagagtgaacaccaagtgaaaattggagacttcggtttaaccaaagcaattgaaaccgataaggagtattacaccgtcaaggatgaccgggacagccctgtgttttggtatgctccagaatgtttaatgcaatctaaattttatattgcctctgacgtctggtcttttggagtcactctgcatgagctgctgacttactgtgattcagattctagtcccatggctttgttcctgaaaatgataggcccaacccatggccagatgacagtcacaagacttgtgaatacgttaaaagaaggaaaacgcctgccgtgcccacctaactgtccagatgaggtttatcaacttatgaggaaatgctgggaattccaaccatccaatcggacaagctttcagaaccttattgaaggatttgaagcacttttaaaataagaagcatgaataacatttaaattccacagattatcaagtccttctcctgcaacaaatgcccaagtcattttttaaaaatttctaatgaaagaagtttgtgttctgtccaaaaagtcactgaactcatacttcagtacatatacatgtataaggcacactgtagtgcttaatatgtgtaaggacttcctctttaaatttggtaccagtaacttagtgacacataatgacaaccaaaatatttgaaagcacttaagcactcctccttgtggaaagaatataccaccatttcatctggctagttcaccatcacaactgcattaccaaaaggggatttttgaaaacgaggagttgaccaaaataatatctgaagatgattgcttttccctgctgccagctgatctgaaatgttttgctggcacattaatcatagataaagaaagattgatggacttagccctcaaatttcagtatctatacagtactagaccatgcattcttaaaatattagataccaggtagtatatattgtttctgtacaaaaatgactgtattctctcaccagtaggacttaaactttgtttctccagtggcttagctcctgttcctttgggtgatcactagcacccatttttgagaaagctggttctacatggggggatagctgtggaatagataatttgctgcatgttaattctcaagaactaagcctgtgccagtgctttcctaagcagtatacctttaatcagaactcattcccagaacctggatgctattacacatgcttttaagaaacgtcaatgtatatccttttataactctaccactttggggcaagctattccagcactggttttgaatgctgtatgcaaccagtctgaataccacatacgctgcactgttcttagagggtttccatacttaccaccgatctacaagggttgatccctgtttttaccatcaatcatcaccctgtggtgcaacacttgaaagacccggctagaggcactatggacttcaggatccactagacagttttcagtttgcttggaggtagctgggtaatcaaaaatgtttagtcattgattcaatgtgaacgattacggtctttatgaccaagagtctgaaaatctttttgttatgctgtttagtattcgtttgatattgttacttttcacctgttgagcccaaattcaggattggttcagtggcagcaatgaagttgccatttaaatttgttcatagcctacatcaccaaggtctctgtgtcaaacctgtggccactctatatgcactttgtttactctttatacaaataaatatactaaagactttacatgca

SEQ ID NO: 8 - DNA, 5115 bp, Homo sapiens
ggggcgggacgggaggcggtgcgtcgctgagcgcaggccgcggcggccgcggagtatcctggagctgcagacagtgcgggcctgcgcccagtcccggctgtcctcgccgcgacccctcctcagccctgggcgcgcgcacgctggggccccgcggggctggccgcctagcgagcctgccggtcgaccccagccagcgcagcgacggggcgctgcctggcccaggcgcacacggaagtgcgcttctctgaagtagctttggaaagtagagaagaaaatccagtttgcttcttggagaacactggacagctgaataaatgcagtatctaaatataaaagaggactgcaatgccatggctttctgtgctaaaatgaggagctccaagaagactgaggtgaacctggaggcccctgagccaggggtggaagtgatcttctatctgtcggacagggagcccctccggctgggcagtggagagtacacagcagaggaactgtgcatcagggctgcacaggcatgccgtatctctcctctttgtcacaacctctttgccctgtatgacgagaacaccaagctctggtatgctccaaatcgcaccatcaccgttgatgacaagatgtccctccggctccactaccggatgaggttctatttcaccaattggcatggaaccaacgacaatgagcagtcagtgtggcgtcattctccaaagaagcagaaaaatggctacgagaaaaaaaagattccagatgcaacccctctccttgatgccagctcactggagtatctgtttgctcagggacagtatgatttggtgaaatgcctggctcctattcgagaccccaagaccgagcaggatggacatgatattgagaacgagtgtctagggatggctgtcctggccatctcacactatgccatgatgaagaagatgcagttgccagaactgcccaaggacatcagctacaagcgatatattccagaaacattgaataagtccatcagacagaggaaccttctcaccaggatgcggataaataatgttttcaaggatttcctaaaggaatttaacaacaagaccatttgtgacagcagcgtgtccacgcatgacctgaaggtgaaatacttggctaccttggaaactttgacaaaacattacggtgctgaaatatttgagacttccatgttactgatttcatcagaaaatgagatgaattggtttcattcgaatgacggtggaaacgttctctactacgaagtgatggtgactgggaatcttggaatccagtggaggcataaaccaaatgttgtttctgttgaaaaggaaaaaaataaactgaagcggaaaaaactggaaaataaacacaagaaggatgaggagaaaaacaagatccgggaagagtggaacaatttttcttacttccctgaaatcactcacattgtaataaaggagtctgtggtcagcattaacaagcaggacaacaagaaaatggaactgaagctctcttcccacgaggaggccttgtcctttgtgtccctggtagatggctacttccggctcacagcagatgcccatcattacctctgcaccgacgtggcccccccgttgatcgtccacaacatacagaatggctgtcatggtccaatctgtacagaatacgccatcaataaattgcggcaagaaggaagcgaggaggggatgtacgtgctgaggtggagctgcaccgactttgacaacatcctcatgaccgtcacctgctttgagaagtctgaggtgcagggtgcccagaagcagttcaagaactttcagatcgaggtgcagaagggccgctacagtctgcacggttcggaccgcagcttccccagcttgggagacctcatgagccacctcaagaagcagatcctgcgcacggataacatcagcttcatgctaaaacgctgctgccagcccaagccccgagaaatctccaacctgctggtggctactaagaaagcccaggagtggcagcccgtctaccccatgagccagctgagtttcgatcggatcctcaagaaggatctggtgcagggcgagcaccttgggagaggcacgagaacacacatctattctgggaccctgatggattacaaggatgacgaaggaacttctgaagagaagaagataaaagtgatcctcaaagtcttagaccccagccacagggatatttccctggccttcttcgaggcagccagcatgatgagacaggtctcccacaaacacatcgtgtacctctatggcgtctgtgtccgcgacgtggagaatatcatggtggaagagtttgtggaagggggtcctctggatctcttcatgcaccggaaaagcgatgtccttaccacaccatggaaattcaaagttgccaaacagctggccagtgccctgagctacttggaggataaagacctggtccatggaaatgtgtgtactaaaaacctcctcctggcccgtgagggcatcgacagtgagtgtggcccattcatcaagctcagtgaccccggcatccccattacggtgctgtctaggcaagaatgcattgaacgaatcccatggattgctcctgagtgtgttgaggactccaagaacctgagtgtggctgctgacaagtggagctttggaaccacgctctgggaaatctgctacaatggcgagatccccttgaaagacaagacgctgattgagaaagagagattctatgaaagccggtgcaggccagtgacaccatcatgtaaggagctggctgacctcatgacccgctgcatgaactatgaccccaatcagaggcctttcttccgagccatcatgagagacattaataagcttgaagagcagaatccagatattgtttcagaaaaaaaaccagcaactgaagtggaccccacacattttgaaaagcgcttcctaaagaggatccgtgacttgggagagggccactttgggaaggttgagctctgcaggtatgaccccgaaggggacaatacaggggagcaggtggctgttaaatctctgaagcctgagagtggaggtaaccacatagctgatctgaaaaaggaaatcgagatcttaaggaacctctatcatgagaacattgtgaagtacaaaggaatctgcacagaagacggaggaaatggtattaagctcatcatggaatttctgccttcgggaagccttaaggaatatcttccaaagaataagaacaaaataaacctcaaacagcagctaaaatatgccgttcagatttgtaaggggatggactatttgggttctcggcaatacgttcaccgggacttggcagcaagaaatgtccttgttgagagtgaacaccaagtgaaaattggagacttcggtttaaccaaagcaattgaaaccgataaggagtattacaccgtcaaggatgaccgggacagccctgtgttttggtatgctccagaatgtttaatgcaatctaaattttatattgcctctgacgtctggtcttttggagtcactctgcatgagctgctgacttactgtgattcagattctagtcccatggctttgttcctgaaaatgataggcccaacccatggccagatgacagtcacaagacttgtgaatacgttaaaagaaggaaaacgcctgccgtgcccacctaactgtccagatgaggtttatcaacttatgaggaaatgctgggaattccaaccatccaatcggacaagctttcagaaccttattgaaggatttgaagcacttttaaaataagaagcatgaataacatttaaattccacagattatcaagtccttctcctgcaacaaatgcccaagtcattttttaaaaatttctaatgaaagaagtttgtgttctgtccaaaaagtcactgaactcatacttcagtacatatacatgtataaggcacactgtagtgcttaatatgtgtaaggacttcctctttaaatttggtaccagtaacttagtgacacataatgacaaccaaaatatttgaaagcacttaagcactcctccttgtggaaagaatataccaccatttcatctggctagttcaccatcacaactgcattaccaaaaggggatttttgaaaacgaggagttgaccaaaataatatctgaagatgattgcttttccctgctgccagctgatctgaaatgttttgctggcacattaatcatagataaagaaagattgatggacttagccctcaaatttcagtatctatacagtactagaccatgcattcttaaaatattagataccaggtagtatatattgtttctgtacaaaaatgactgtattctctcaccagtaggacttaaactttgtttctccagtggcttagctcctgttcctttgggtgatcactagcacccatttttgagaaagctggttctacatggggggatagctgtggaatagataatttgctgcatgttaattctcaagaactaagcctgtgccagtgctttcctaagcagtatacctttaatcagaactcattcccagaacctggatgctattacacatgcttttaagaaacgtcaatgtatatccttttataactctaccactttggggcaagctattccagcactggttttgaatgctgtatgcaaccagtctgaataccacatacgctgcactgttcttagagggtttccatacttaccaccgatctacaagggttgatccctgtttttaccatcaatcatcaccctgtggtgcaacacttgaaagacccggctagaggcactatggacttcaggatccactagacagttttcagtttgcttggaggtagctgggtaatcaaaaatgtttagtcattgattcaatgtgaacgattacggtctttatgaccaagagtctgaaaatctttttgttatgctgtttagtattcgtttgatattgttacttttcacctgttgagcccaaattcaggattggttcagtggcagcaatgaagttgccatttaaatttgttcatagcctacatcaccaaggtctctgtgtcaaacctgtggccactctatatgcactttgtttactctttatacaaataaatatactaaagactttacatgca

SEQ ID NO: 9 - DNA, 5285 bp, Homo sapiens
ctgcaggaaggagagaggaagaggagcagaagggggcagcagcggacgccgctaacggcctccctcggcgctgacaggctgggccggcgcccggctcgcttgggtgttcgcgtcgccacttcggcttctcggccggtcgggcccctcggcccgggcttgcggcgcgcgtcggggctgagggctgctgcggcgcagggagaggcctggtcctcgctgccgagggatgtgagtgggagctgagcccacactggagggcccccgagggcccagcctggaggtcgttcagagccgtgcccgtcccggggcttcgcagaccttgacccgccgggtaggagccgcccctgcgggctcgagggcgcgctctggtcgcccgatctgtgtagccggtttcagaagcaggcaacaggaacaagatgtgaactgtttctcttctgcagaaaaagaggctcttcctcctcctcccgcgacggcaaatgttctgaaaaagactctgcatgggaatggcctgccttacgatgacagaaatggagggaacatccacctcttctatatatcagaatggtgatatttctggaaatgccaattctatgaagcaaatagatccagttcttcaggtgtatctttaccattcccttgggaaatctgaggcagattatctgacctttccatctggggagtatgttgcagaagaaatctgtattgctgcttctaaagcttgtggtatcacacctgtgtatcataatatgtttgctttaatgagtgaaacagaaaggatctggtatccacccaaccatgtcttccatatagatgagtcaaccaggcataatgtactctacagaataagattttactttcctcgttggtattgcagtggcagcaacagagcctatcggcatggaatatctcgaggtgctgaagctcctcttcttgatgactttgtcatgtcttacctctttgctcagtggcggcatgattttgtgcacggatggataaaagtacctgtgactcatgaaacacaggaagaatgtcttgggatggcagtgttagatatgatgagaatagccaaagaaaacgatcaaaccccactggccatctataactctatcagctacaagacattcttaccaaaatgtattcgagcaaagatccaagactatcatattttgacaaggaagcgaataaggtacagatttcgcagatttattcagcaattcagccaatgcaaagccactgccagaaacttgaaacttaagtatcttataaatctggaaactctgcagtctgccttctacacagagaaatttgaagtaaaagaacctggaagtggtccttcaggtgaggagatttttgcaaccattataataactggaaacggtggaattcagtggtcaagagggaaacataaagaaagtgagacactgacagaacaggatttacagttatattgcgattttcctaatattattgatgtcagtattaagcaagcaaaccaagagggttcaaatgaaagccgagttgtaactatccataagcaagatggtaaaaatctggaaattgaacttagctcattaagggaagctttgtctttcgtgtcattaattgatggatattatagattaactgcagatgcacatcattacctctgtaaagaagtagcacctccagccgtgcttgaaaatatacaaagcaactgtcatggcccaatttcgatggattttgccattagtaaactgaagaaagcaggtaatcagactggactgtatgtacttcgatgcagtcctaaggactttaataaatattttttgacttttgctgtcgagcgagaaaatgtcattgaatataaacactgtttgattacaaaaaatgagaatgaagagtacaacctcagtgggacaaagaagaacttcagcagtcttaaagatcttttgaattgttaccagatggaaactgttcgctcagacaatataattttccagtttactaaatgctgtcccccaaagccaaaagataaatcaaaccttctagtcttcagaacgaatggtgtttctgatgtaccaacctcaccaacattacagaggcctactcatatgaaccaaatggtgtttcacaaaatcagaaatgaagatttgatatttaatgaaagccttggccaaggcacttttacaaagatttttaaaggcgtacgaagagaagtaggagactacggtcaactgcatgaaacagaagttcttttaaaagttctggataaagcacacagaaactattcagagtctttctttgaagcagcaagtatgatgagcaagctttctcacaagcatttggttttaaattatggagtatgtgtctgtggagacgagaatattctggttcaggagtttgtaaaatttggatcactagatacatatctgaaaaagaataaaaattgtataaatatattatggaaacttgaagttgctaaacagttggcatgggccatgcattttctagaagaaaacacccttattcatgggaatgtatgtgccaaaaatattctgcttatcagagaagaagacaggaagacaggaaatcctcctttcatcaaacttagtgatcctggcattagtattacagttttgccaaaggacattcttcaggagagaataccatgggtaccacctgaatgcattgaaaatcctaaaaatttaaatttggcaacagacaaatggagttttggtaccactttgtgggaaatctgcagtggaggagataaacctctaagtgctctggattctcaaagaaagctacaattttatgaagataggcatcagcttcctgcaccaaagtgggcagaattagcaaaccttataaataattgtatggattatgaaccagatttcaggccttctttcagagccatcatacgagatcttaacagtttgtttactccagattatgaactattaacagaaaatgacatgttaccaaatatgaggataggtgccctggggttttctggtgcctttgaagaccgggatcctacacagtttgaagagagacatttgaaatttctacagcaacttggcaagggtaattttgggagtgtggagatgtgccggtatgaccctctacaggacaacactggggaggtggtcgctgtaaaaaagcttcagcatagtactgaagagcacctaagagactttgaaagggaaattgaaatcctgaaatccctacagcatgacaacattgtaaagtacaagggagtgtgctacagtgctggtcggcgtaatctaaaattaattatggaatatttaccatatggaagtttacgagactatcttcaaaaacataaagaacggatagatcacataaaacttctgcagtacacatctcagatatgcaagggtatggagtatcttggtacaaaaaggtatatccacagggatctggcaacgagaaatatattggtggagaacgagaacagagttaaaattggagattttgggttaaccaaagtcttgccacaagacaaagaatactataaagtaaaagaacctggtgaaagtcccatattctggtatgctccagaatcactgacagagagcaagttttctgtggcctcagatgtttggagctttggagtggttctgtatgaacttttcacatacattgagaagagtaaaagtccaccagcggaatttatgcgtatgattggcaatgacaaacaaggacagatgatcgtgttccatttgatagaacttttgaagaataatggaagattaccaagaccagatggatgcccagatgagatctatatgatcatgacagaatgctggaacaataatgtaaatcaacgcccctcctttagggatctagctcttcgagtggatcaaataagggataacatggctggatgaaagaaatgaccttcattctgagaccaaagtagatttacagaacaaagttttatatttcacattgctgtggactattattacatatatcattattatataaatcatgatgctagccagcaaagatgtgaaaatatctgctcaaaactttcaaagtttagtaagtttttcttcatgaggccaccagtaaaagacattaatgagaattccttagcaaggattttgtaagaagtttcttaaacattgtcagttaacatcactcttgtctggcaaaagaaaaaaaatagactttttcaactcagctttttgagacctgaaaaaattattatgtaaattttgcaatgttaaagatgcacagaatatgtatgtatagtttttaccacagtggatgtataataccttggcatcttgtgtgatgttttacacacatgagggctggtgttcattaatactgttttctaatttttccatagttaatctataattaattacttcactatacaaacaaattaagatgttcagataattgaataagtacctttgtgtccttgttcatttatatcgctggccagcattataagcaggtgtatacttttagcttgtagttccatgtactgtaaatatttttcacataaagggaacaaatgtctagttttatttgtataggaaatttccctgaccctaaataatacattttgaaatgaaacaagcttacaaagatataatctattttattatggtttcccttgtatctatttgtggtgaatgtgttttttaaatggaactatctccaaatttttctaagactactatgaacagttttcttttaaaattttgagattaagaatgccaggaatattgtcatcctttgagctgctgactgccaataacattcttcgatctctgggatttatgctcatgaactaaatttaagcttaagccataaaatagattagattgttttttaaaaatggatagctcattaagaagtgcagcaggttaagaattttttcctaaagactgtatatttgaggggtttcagaattttgcattgcagtcatagaagagatttatttcctttttagaggggaaatgaggtaaataagtaaaaaagtatgcttgttaattttattcaagaatgccagtagaaaattcataacgtgtatctttaagaaaaatgagcatacatcttaaatcttttcaattaagtataaggggttgttcgttgttgtcatttgttatagtgctactccactttagacaccatagctaaaataaaatatggtgggttttgtgtgtgtgtgtgtgtgtgtgtgtgtgtgtgtgtgtgtgttatttatacaaaacttaaaatacttgctgttttgattaaaaagaaaatagtttcttacttta

SEQ ID NO: 10 - DNA, 5386 bp, Homo sapiens
attcggggagactgcaggccaaccgggaggctgagttcgaagctagcagggcggcgaagccagtgtcgcccgcggcgttgagaagacggtgtggccccggagagggtggagacaactgtgacgggcttcccggctgcccgaagtgggagtggtgtggggctgcaggaaggagagaggaagaggagcagaagggggcagcagcggacgccgctaacggcctccctcggcgctgacaggctgggccggcgcccggctcgcttgggtgttcgcgtcgccacttcggcttctcggccggtcgggcccctcggcccgggcttgcggcgcgcgtcggggctgagggctgctgcggcgcagggagaggcctggtcctcgctgccgagggatgtgagtgggagctgagcccacactggagggcccccgagggcccagcctggaggtcgttcagagccgtgcccgtcccggggcttcgcagaccttgacccgccgggtttcagaagcaggcaacaggaacaagatgtgaactgtttctcttctgcagaaaaagaggctcttcctcctcctcccgcgacggcaaatgttctgaaaaagactctgcatgggaatggcctgccttacgatgacagaaatggagggaacatccacctcttctatatatcagaatggtgatatttctggaaatgccaattctatgaagcaaatagatccagttcttcaggtgtatctttaccattcccttgggaaatctgaggcagattatctgacctttccatctggggagtatgttgcagaagaaatctgtattgctgcttctaaagcttgtggtatcacacctgtgtatcataatatgtttgctttaatgagtgaaacagaaaggatctggtatccacccaaccatgtcttccatatagatgagtcaaccaggcataatgtactctacagaataagattttactttcctcgttggtattgcagtggcagcaacagagcctatcggcatggaatatctcgaggtgctgaagctcctcttcttgatgactttgtcatgtcttacctctttgctcagtggcggcatgattttgtgcacggatggataaaagtacctgtgactcatgaaacacaggaagaatgtcttgggatggcagtgttagatatgatgagaatagccaaagaaaacgatcaaaccccactggccatctataactctatcagctacaagacattcttaccaaaatgtattcgagcaaagatccaagactatcatattttgacaaggaagcgaataaggtacagatttcgcagatttattcagcaattcagccaatgcaaagccactgccagaaacttgaaacttaagtatcttataaatctggaaactctgcagtctgccttctacacagagaaatttgaagtaaaagaacctggaagtggtccttcaggtgaggagatttttgcaaccattataataactggaaacggtggaattcagtggtcaagagggaaacataaagaaagtgagacactgacagaacaggatttacagttatattgcgattttcctaatattattgatgtcagtattaagcaagcaaaccaagagggttcaaatgaaagccgagttgtaactatccataagcaagatggtaaaaatctggaaattgaacttagctcattaagggaagctttgtctttcgtgtcattaattgatggatattatagattaactgcagatgcacatcattacctctgtaaagaagtagcacctccagccgtgcttgaaaatatacaaagcaactgtcatggcccaatttcgatggattttgccattagtaaactgaagaaagcaggtaatcagactggactgtatgtacttcgatgcagtcctaaggactttaataaatattttttgacttttgctgtcgagcgagaaaatgtcattgaatataaacactgtttgattacaaaaaatgagaatgaagagtacaacctcagtgggacaaagaagaacttcagcagtcttaaagatcttttgaattgttaccagatggaaactgttcgctcagacaatataattttccagtttactaaatgctgtcccccaaagccaaaagataaatcaaaccttctagtcttcagaacgaatggtgtttctgatgtaccaacctcaccaacattacagaggcctactcatatgaaccaaatggtgtttcacaaaatcagaaatgaagatttgatatttaatgaaagccttggccaaggcacttttacaaagatttttaaaggcgtacgaagagaagtaggagactacggtcaactgcatgaaacagaagttcttttaaaagttctggataaagcacacagaaactattcagagtctttctttgaagcagcaagtatgatgagcaagctttctcacaagcatttggttttaaattatggagtatgtgtctgtggagacgagaatattctggttcaggagtttgtaaaatttggatcactagatacatatctgaaaaagaataaaaattgtataaatatattatggaaacttgaagttgctaaacagttggcatgggccatgcattttctagaagaaaacacccttattcatgggaatgtatgtgccaaaaatattctgcttatcagagaagaagacaggaagacaggaaatcctcctttcatcaaacttagtgatcctggcattagtattacagttttgccaaaggacattcttcaggagagaataccatgggtaccacctgaatgcattgaaaatcctaaaaatttaaatttggcaacagacaaatggagttttggtaccactttgtgggaaatctgcagtggaggagataaacctctaagtgctctggattctcaaagaaagctacaattttatgaagataggcatcagcttcctgcaccaaagtgggcagaattagcaaaccttataaataattgtatggattatgaaccagatttcaggccttctttcagagccatcatacgagatcttaacagtttgtttactccagattatgaactattaacagaaaatgacatgttaccaaatatgaggataggtgccctggggttttctggtgcctttgaagaccgggatcctacacagtttgaagagagacatttgaaatttctacagcaacttggcaagggtaattttgggagtgtggagatgtgccggtatgaccctctacaggacaacactggggaggtggtcgctgtaaaaaagcttcagcatagtactgaagagcacctaagagactttgaaagggaaattgaaatcctgaaatccctacagcatgacaacattgtaaagtacaagggagtgtgctacagtgctggtcggcgtaatctaaaattaattatggaatatttaccatatggaagtttacgagactatcttcaaaaacataaagaacggatagatcacataaaacttctgcagtacacatctcagatatgcaagggtatggagtatcttggtacaaaaaggtatatccacagggatctggcaacgagaaatatattggtggagaacgagaacagagttaaaattggagattttgggttaaccaaagtcttgccacaagacaaagaatactataaagtaaaagaacctggtgaaagtcccatattctggtatgctccagaatcactgacagagagcaagttttctgtggcctcagatgtttggagctttggagtggttctgtatgaacttttcacatacattgagaagagtaaaagtccaccagcggaatttatgcgtatgattggcaatgacaaacaaggacagatgatcgtgttccatttgatagaacttttgaagaataatggaagattaccaagaccagatggatgcccagatgagatctatatgatcatgacagaatgctggaacaataatgtaaatcaacgcccctcctttagggatctagctcttcgagtggatcaaataagggataacatggctggatgaaagaaatgaccttcattctgagaccaaagtagatttacagaacaaagttttatatttcacattgctgtggactattattacatatatcattattatataaatcatgatgctagccagcaaagatgtgaaaatatctgctcaaaactttcaaagtttagtaagtttttcttcatgaggccaccagtaaaagacattaatgagaattccttagcaaggattttgtaagaagtttcttaaacattgtcagttaacatcactcttgtctggcaaaagaaaaaaaatagactttttcaactcagctttttgagacctgaaaaaattattatgtaaattttgcaatgttaaagatgcacagaatatgtatgtatagtttttaccacagtggatgtataataccttggcatcttgtgtgatgttttacacacatgagggctggtgttcattaatactgttttctaatttttccatagttaatctataattaattacttcactatacaaacaaattaagatgttcagataattgaataagtacctttgtgtccttgttcatttatatcgctggccagcattataagcaggtgtatacttttagcttgtagttccatgtactgtaaatatttttcacataaagggaacaaatgtctagttttatttgtataggaaatttccctgaccctaaataatacattttgaaatgaaacaagcttacaaagatataatctattttattatggtttcccttgtatctatttgtggtgaatgtgttttttaaatggaactatctccaaatttttctaagactactatgaacagttttcttttaaaattttgagattaagaatgccaggaatattgtcatcctttgagctgctgactgccaataacattcttcgatctctgggatttatgctcatgaactaaatttaagcttaagccataaaatagattagattgttttttaaaaatggatagctcattaagaagtgcagcaggttaagaattttttcctaaagactgtatatttgaggggtttcagaattttgcattgcagtcatagaagagatttatttcctttttagaggggaaatgaggtaaataagtaaaaaagtatgcttgttaattttattcaagaatgccagtagaaaattcataacgtgtatctttaagaaaaatgagcatacatcttaaatcttttcaattaagtataaggggttgttcgttgttgtcatttgttatagtgctactccactttagacaccatagctaaaataaaatatggtgggttttgtgtgtgtgtgtgtgtgtgtgtgtgtgtgtgtgtgtgtgttatttatacaaaacttaaaatacttgctgttttgattaaaaagaaaatagtttcttacttta

SEQ ID NO: 11 - DNA, 4904 bp, Homo sapiens
attcggggagactgcaggccaaccgggaggctgagttcgaagctagcagggcggcgaagccagtgtcgcccgcggcgttgagaagacggcaaatgttctgaaaaagactctgcatgggaatggcctgccttacgatgacagaaatggagggaacatccacctcttctatatatcagaatggtgatatttctggaaatgccaattctatgaagcaaatagatccagttcttcaggtgtatctttaccattcccttgggaaatctgaggcagattatctgacctttccatctggggagtatgttgcagaagaaatctgtattgctgcttctaaagcttgtggtatcacacctgtgtatcataatatgtttgctttaatgagtgaaacagaaaggatctggtatccacccaaccatgtcttccatatagatgagtcaaccaggcataatgtactctacagaataagattttactttcctcgttggtattgcagtggcagcaacagagcctatcggcatggaatatctcgaggtgctgaagctcctcttcttgatgactttgtcatgtcttacctctttgctcagtggcggcatgattttgtgcacggatggataaaagtacctgtgactcatgaaacacaggaagaatgtcttgggatggcagtgttagatatgatgagaatagccaaagaaaacgatcaaaccccactggccatctataactctatcagctacaagacattcttaccaaaatgtattcgagcaaagatccaagactatcatattttgacaaggaagcgaataaggtacagatttcgcagatttattcagcaattcagccaatgcaaagccactgccagaaacttgaaacttaagtatcttataaatctggaaactctgcagtctgccttctacacagagaaatttgaagtaaaagaacctggaagtggtccttcaggtgaggagatttttgcaaccattataataactggaaacggtggaattcagtggtcaagagggaaacataaagaaagtgagacactgacagaacaggatttacagttatattgcgattttcctaatattattgatgtcagtattaagcaagcaaaccaagagggttcaaatgaaagccgagttgtaactatccataagcaagatggtaaaaatctggaaattgaacttagctcattaagggaagctttgtctttcgtgtcattaattgatggatattatagattaactgcagatgcacatcattacctctgtaaagaagtagcacctccagccgtgcttgaaaatatacaaagcaactgtcatggcccaatttcgatggattttgccattagtaaactgaagaaagcaggtaatcagactggactgtatgtacttcgatgcagtcctaaggactttaataaatattttttgacttttgctgtcgagcgagaaaatgtcattgaatataaacactgtttgattacaaaaaatgagaatgaagagtacaacctcagtgggacaaagaagaacttcagcagtcttaaagatcttttgaattgttaccagatggaaactgttcgctcagacaatataattttccagtttactaaatgctgtcccccaaagccaaaagataaatcaaaccttctagtcttcagaacgaatggtgtttctgatgtaccaacctcaccaacattacagaggcctactcatatgaaccaaatggtgtttcacaaaatcagaaatgaagatttgatatttaatgaaagccttggccaaggcacttttacaaagatttttaaaggcgtacgaagagaagtaggagactacggtcaactgcatgaaacagaagttcttttaaaagttctggataaagcacacagaaactattcagagtctttctttgaagcagcaagtatgatgagcaagctttctcacaagcatttggttttaaattatggagtatgtgtctgtggagacgagaatattctggttcaggagtttgtaaaatttggatcactagatacatatctgaaaaagaataaaaattgtataaatatattatggaaacttgaagttgctaaacagttggcatgggccatgcattttctagaagaaaacacccttattcatgggaatgtatgtgccaaaaatattctgcttatcagagaagaagacaggaagacaggaaatcctcctttcatcaaacttagtgatcctggcattagtattacagttttgccaaaggacattcttcaggagagaataccatgggtaccacctgaatgcattgaaaatcctaaaaatttaaatttggcaacagacaaatggagttttggtaccactttgtgggaaatctgcagtggaggagataaacctctaagtgctctggattctcaaagaaagctacaattttatgaagataggcatcagcttcctgcaccaaagtgggcagaattagcaaaccttataaataattgtatggattatgaaccagatttcaggccttctttcagagccatcatacgagatcttaacagtttgtttactccagattatgaactattaacagaaaatgacatgttaccaaatatgaggataggtgccctggggttttctggtgcctttgaagaccgggatcctacacagtttgaagagagacatttgaaatttctacagcaacttggcaagggtaattttgggagtgtggagatgtgccggtatgaccctctacaggacaacactggggaggtggtcgctgtaaaaaagcttcagcatagtactgaagagcacctaagagactttgaaagggaaattgaaatcctgaaatccctacagcatgacaacattgtaaagtacaagggagtgtgctacagtgctggtcggcgtaatctaaaattaattatggaatatttaccatatggaagtttacgagactatcttcaaaaacataaagaacggatagatcacataaaacttctgcagtacacatctcagatatgcaagggtatggagtatcttggtacaaaaaggtatatccacagggatctggcaacgagaaatatattggtggagaacgagaacagagttaaaattggagattttgggttaaccaaagtcttgccacaagacaaagaatactataaagtaaaagaacctggtgaaagtcccatattctggtatgctccagaatcactgacagagagcaagttttctgtggcctcagatgtttggagctttggagtggttctgtatgaacttttcacatacattgagaagagtaaaagtccaccagcggaatttatgcgtatgattggcaatgacaaacaaggacagatgatcgtgttccatttgatagaacttttgaagaataatggaagattaccaagaccagatggatgcccagatgagatctatatgatcatgacagaatgctggaacaataatgtaaatcaacgcccctcctttagggatctagctcttcgagtggatcaaataagggataacatggctggatgaaagaaatgaccttcattctgagaccaaagtagatttacagaacaaagttttatatttcacattgctgtggactattattacatatatcattattatataaatcatgatgctagccagcaaagatgtgaaaatatctgctcaaaactttcaaagtttagtaagtttttcttcatgaggccaccagtaaaagacattaatgagaattccttagcaaggattttgtaagaagtttcttaaacattgtcagttaacatcactcttgtctggcaaaagaaaaaaaatagactttttcaactcagctttttgagacctgaaaaaattattatgtaaattttgcaatgttaaagatgcacagaatatgtatgtatagtttttaccacagtggatgtataataccttggcatcttgtgtgatgttttacacacatgagggctggtgttcattaatactgttttctaatttttccatagttaatctataattaattacttcactatacaaacaaattaagatgttcagataattgaataagtacctttgtgtccttgttcatttatatcgctggccagcattataagcaggtgtatacttttagcttgtagttccatgtactgtaaatatttttcacataaagggaacaaatgtctagttttatttgtataggaaatttccctgaccctaaataatacattttgaaatgaaacaagcttacaaagatataatctattttattatggtttcccttgtatctatttgtggtgaatgtgttttttaaatggaactatctccaaatttttctaagactactatgaacagttttcttttaaaattttgagattaagaatgccaggaatattgtcatcctttgagctgctgactgccaataacattcttcgatctctgggatttatgctcatgaactaaatttaagcttaagccataaaatagattagattgttttttaaaaatggatagctcattaagaagtgcagcaggttaagaattttttcctaaagactgtatatttgaggggtttcagaattttgcattgcagtcatagaagagatttatttcctttttagaggggaaatgaggtaaataagtaaaaaagtatgcttgttaattttattcaagaatgccagtagaaaattcataacgtgtatctttaagaaaaatgagcatacatcttaaatcttttcaattaagtataaggggttgttcgttgttgtcatttgttatagtgctactccactttagacaccatagctaaaataaaatatggtgggttttgtgtgtgtgtgtgtgtgtgtgtgtgtgtgtgtgtgtgtgttatttatacaaaacttaaaatacttgctgttttgattaaaaagaaaatagtttcttacttta

SEQ ID NO: 12 - DNA, 5217 bp, Homo sapiens
gggagtggtgtggggctgcaggaaggagagaggaagaggagcagaagggggcagcagcggacgccgctaacggcctccctcggcgctgacaggctgggccggcgcccggctcgcttgggtgttcgcgtcgccacttcggcttctcggccggtcgggcccctcggcccgggcttgcggcgcgcgtcggggctgagggctgctgcggcgcagggagaggcctggtcctcgctgccgagggatgtgagtgggagctgagcccacactggagggcccccgagggcccagcctggaggtcgttcagagccgtgcccgtcccggggcttcgcagaccttgacccgccgggtaggagccgcccctgcgggctcgagggcgcgctctggtcgcccgatctgtgtagccggcaaatgttctgaaaaagactctgcatgggaatggcctgccttacgatgacagaaatggagggaacatccacctcttctatatatcagaatggtgatatttctggaaatgccaattctatgaagcaaatagatccagttcttcaggtgtatctttaccattcccttgggaaatctgaggcagattatctgacctttccatctggggagtatgttgcagaagaaatctgtattgctgcttctaaagcttgtggtatcacacctgtgtatcataatatgtttgctttaatgagtgaaacagaaaggatctggtatccacccaaccatgtcttccatatagatgagtcaaccaggcataatgtactctacagaataagattttactttcctcgttggtattgcagtggcagcaacagagcctatcggcatggaatatctcgaggtgctgaagctcctcttcttgatgactttgtcatgtcttacctctttgctcagtggcggcatgattttgtgcacggatggataaaagtacctgtgactcatgaaacacaggaagaatgtcttgggatggcagtgttagatatgatgagaatagccaaagaaaacgatcaaaccccactggccatctataactctatcagctacaagacattcttaccaaaatgtattcgagcaaagatccaagactatcatattttgacaaggaagcgaataaggtacagatttcgcagatttattcagcaattcagccaatgcaaagccactgccagaaacttgaaacttaagtatcttataaatctggaaactctgcagtctgccttctacacagagaaatttgaagtaaaagaacctggaagtggtccttcaggtgaggagatttttgcaaccattataataactggaaacggtggaattcagtggtcaagagggaaacataaagaaagtgagacactgacagaacaggatttacagttatattgcgattttcctaatattattgatgtcagtattaagcaagcaaaccaagagggttcaaatgaaagccgagttgtaactatccataagcaagatggtaaaaatctggaaattgaacttagctcattaagggaagctttgtctttcgtgtcattaattgatggatattatagattaactgcagatgcacatcattacctctgtaaagaagtagcacctccagccgtgcttgaaaatatacaaagcaactgtcatggcccaatttcgatggattttgccattagtaaactgaagaaagcaggtaatcagactggactgtatgtacttcgatgcagtcctaaggactttaataaatattttttgacttttgctgtcgagcgagaaaatgtcattgaatataaacactgtttgattacaaaaaatgagaatgaagagtacaacctcagtgggacaaagaagaacttcagcagtcttaaagatcttttgaattgttaccagatggaaactgttcgctcagacaatataattttccagtttactaaatgctgtcccccaaagccaaaagataaatcaaaccttctagtcttcagaacgaatggtgtttctgatgtaccaacctcaccaacattacagaggcctactcatatgaaccaaatggtgtttcacaaaatcagaaatgaagatttgatatttaatgaaagccttggccaaggcacttttacaaagatttttaaaggcgtacgaagagaagtaggagactacggtcaactgcatgaaacagaagttcttttaaaagttctggataaagcacacagaaactattcagagtctttctttgaagcagcaagtatgatgagcaagctttctcacaagcatttggttttaaattatggagtatgtgtctgtggagacgagaatattctggttcaggagtttgtaaaatttggatcactagatacatatctgaaaaagaataaaaattgtataaatatattatggaaacttgaagttgctaaacagttggcatgggccatgcattttctagaagaaaacacccttattcatgggaatgtatgtgccaaaaatattctgcttatcagagaagaagacaggaagacaggaaatcctcctttcatcaaacttagtgatcctggcattagtattacagttttgccaaaggacattcttcaggagagaataccatgggtaccacctgaatgcattgaaaatcctaaaaatttaaatttggcaacagacaaatggagttttggtaccactttgtgggaaatctgcagtggaggagataaacctctaagtgctctggattctcaaagaaagctacaattttatgaagataggcatcagcttcctgcaccaaagtgggcagaattagcaaaccttataaataattgtatggattatgaaccagatttcaggccttctttcagagccatcatacgagatcttaacagtttgtttactccagattatgaactattaacagaaaatgacatgttaccaaatatgaggataggtgccctggggttttctggtgcctttgaagaccgggatcctacacagtttgaagagagacatttgaaatttctacagcaacttggcaagggtaattttgggagtgtggagatgtgccggtatgaccctctacaggacaacactggggaggtggtcgctgtaaaaaagcttcagcatagtactgaagagcacctaagagactttgaaagggaaattgaaatcctgaaatccctacagcatgacaacattgtaaagtacaagggagtgtgctacagtgctggtcggcgtaatctaaaattaattatggaatatttaccatatggaagtttacgagactatcttcaaaaacataaagaacggatagatcacataaaacttctgcagtacacatctcagatatgcaagggtatggagtatcttggtacaaaaaggtatatccacagggatctggcaacgagaaatatattggtggagaacgagaacagagttaaaattggagattttgggttaaccaaagtcttgccacaagacaaagaatactataaagtaaaagaacctggtgaaagtcccatattctggtatgctccagaatcactgacagagagcaagttttctgtggcctcagatgtttggagctttggagtggttctgtatgaacttttcacatacattgagaagagtaaaagtccaccagcggaatttatgcgtatgattggcaatgacaaacaaggacagatgatcgtgttccatttgatagaacttttgaagaataatggaagattaccaagaccagatggatgcccagatgagatctatatgatcatgacagaatgctggaacaataatgtaaatcaacgcccctcctttagggatctagctcttcgagtggatcaaataagggataacatggctggatgaaagaaatgaccttcattctgagaccaaagtagatttacagaacaaagttttatatttcacattgctgtggactattattacatatatcattattatataaatcatgatgctagccagcaaagatgtgaaaatatctgctcaaaactttcaaagtttagtaagtttttcttcatgaggccaccagtaaaagacattaatgagaattccttagcaaggattttgtaagaagtttcttaaacattgtcagttaacatcactcttgtctggcaaaagaaaaaaaatagactttttcaactcagctttttgagacctgaaaaaattattatgtaaattttgcaatgttaaagatgcacagaatatgtatgtatagtttttaccacagtggatgtataataccttggcatcttgtgtgatgttttacacacatgagggctggtgttcattaatactgttttctaatttttccatagttaatctataattaattacttcactatacaaacaaattaagatgttcagataattgaataagtacctttgtgtccttgttcatttatatcgctggccagcattataagcaggtgtatacttttagcttgtagttccatgtactgtaaatatttttcacataaagggaacaaatgtctagttttatttgtataggaaatttccctgaccctaaataatacattttgaaatgaaacaagcttacaaagatataatctattttattatggtttcccttgtatctatttgtggtgaatgtgttttttaaatggaactatctccaaatttttctaagactactatgaacagttttcttttaaaattttgagattaagaatgccaggaatattgtcatcctttgagctgctgactgccaataacattcttcgatctctgggatttatgctcatgaactaaatttaagcttaagccataaaatagattagattgttttttaaaaatggatagctcattaagaagtgcagcaggttaagaattttttcctaaagactgtatatttgaggggtttcagaattttgcattgcagtcatagaagagatttatttcctttttagaggggaaatgaggtaaataagtaaaaaagtatgcttgttaattttattcaagaatgccagtagaaaattcataacgtgtatctttaagaaaaatgagcatacatcttaaatcttttcaattaagtataaggggttgttcgttgttgtcatttgttatagtgctactccactttagacaccatagctaaaataaaatatggtgggttttgtgtgtgtgtgtgtgtgtgtgtgtgtgtgtgtgtgtgtgttatttatacaaaacttaaaatacttgctgttttgattaaaaagaaaatagtttcttacttta

SEQ ID NO: 13 - DNA, 5449 bp, Homo sapiens
cacacaggaaggagccgagtgggactttcctctcgctgcctcccggctctgcccgcccttcgaaagtccagggtccctgcccgctaggcaagttgcactcatggcacctccaagtgaagagacgcccctgatccctcagcgttcatgcagcctcttgtccacggaggctggtgccctgcatgtgctgctgcccgctcggggccccgggcccccccagcgcctatctttctcctttggggaccacttggctgaggacctgtgcgtgcaggctgccaaggccagcggcatcctgcctgtgtaccactccctctttgctctggccacggaggacctgtcctgctggttccccccgagccacatcttctccgtggaggatgccagcacccaagtcctgctgtacaggattcgcttttacttccccaattggtttgggctggagaagtgccaccgcttcgggctacgcaaggatttggccagtgctatccttgacctgccagtcctggagcacctctttgcccagcaccgcagtgacctggtgagtgggcgcctccccgtgggcctcagtctcaaggagcagggtgagtgtctcagcctggccgtgttggacctggcccggatggcgcgagagcaggcccagcggccgggagagctgctgaagactgtcagctacaaggcctgcctacccccaagcctgcgcgacctgatccagggcctgagcttcgtgacgcggaggcgtattcggaggacggtgcgcagagccctgcgccgcgtggccgcctgccaggcagaccggcactcgctcatggccaagtacatcatggacctggagcggctggatccagccggggccgccgagaccttccacgtgggcctccctggggcccttggtggccacgacgggctggggctgctccgcgtggctggtgacggcggcatcgcctggacccagggagaacaggaggtcctccagcccttctgcgactttccagaaatcgtagacattagcatcaagcaggccccgcgcgttggcccggccggagagcaccgcctggtcactgttaccaggacagacaaccagattttagaggccgagttcccagggctgcccgaggctctgtcgttcgtggcgctcgtggacggctacttccggctgaccacggactcccagcacttcttctgcaaggaggtggcaccgccgaggctgctggaggaagtggccgagcagtgccacggccccatcactctggactttgccatcaacaagctcaagactgggggctcacgtcctggctcctatgttctccgccgcagcccccaggactttgacagcttcctcctcactgtctgtgtccagaacccccttggtcctgattataagggctgcctcatccggcgcagccccacaggaaccttccttctggttggcctcagccgaccccacagcagtcttcgagagctcctggcaacctgctgggatggggggctgcacgtagatggggtggcagtgaccctcacttcctgctgtatccccagacccaaagaaaagtccaacctgatcgtggtccagagaggtcacagcccacccacatcatccttggttcagccccaatcccaataccagctgagtcagatgacatttcacaagatccctgctgacagcctggagtggcatgagaacctgggccatgggtccttcaccaagatttaccggggctgtcgccatgaggtggtggatggggaggcccgaaagacagaggtgctgctgaaggtcatggatgccaagcacaagaactgcatggagtcattcctggaagcagcgagcttgatgagccaagtgtcgtaccggcatctcgtgctgctccacggcgtgtgcatggctggagacagcaccatggtgcaggaatttgtacacctgggggccatagacatgtatctgcgaaaacgtggccacctggtgccagccagctggaagctgcaggtggtcaaacagctggcctacgccctcaactatctggaggacaaaggcctgccccatggcaatgtctctgcccggaaggtgctcctggctcgggagggggctgatgggagcccgcccttcatcaagctgagtgaccctggggtcagccccgctgtgttaagcctggagatgctcaccgacaggatcccctgggtggcccccgagtgtctccgggaggcgcagacacttagcttggaagctgacaagtggggcttcggcgccacggtctgggaagtgtttagtggcgtcaccatgcccatcagtgccctggatcctgctaagaaactccaattttatgaggaccggcagcagctgccggcccccaagtggacagagctggccctgctgattcaacagtgcatggcctatgagccggtccagaggccctccttccgagccgtcattcgtgacctcaatagcctcatctcttcagactatgagctcctctcagaccccacacctggtgccctggcacctcgtgatgggctgtggaatggtgcccagctctatgcctgccaagaccccacgatcttcgaggagagacacctcaagtacatctcacagctgggcaagggcaactttggcagcgtggagctgtgccgctatgacccgctaggcgacaatacaggtgccctggtggccgtgaaacagctgcagcacagcgggccagaccagcagagggactttcagcgggagattcagatcctcaaagcactgcacagtgatttcattgtcaagtatcgtggtgtcagctatggcccgggccgccagagcctgcggctggtcatggagtacctgcccagcggctgcttgcgcgacttcctgcagcggcaccgcgcgcgcctcgatgccagccgcctccttctctattcctcgcagatctgcaagggcatggagtacctgggctcccgccgctgcgtgcaccgcgacctggccgcccgaaacatcctcgtggagagcgaggcacacgtcaagatcgctgacttcggcctagctaagctgctgccgcttgacaaagactactacgtggtccgcgagccaggccagagccccattttctggtatgcccccgaatccctctcggacaacatcttctctcgccagtcagacgtctggagcttcggggtcgtcctgtacgagctcttcacctactgcgacaaaagctgcagcccctcggccgagttcctgcggatgatgggatgtgagcgggatgtccccgccctctgccgcctcttggaactgctggaggagggccagaggctgccggcgcctcctgcctgccctgctgaggttcacgagctcatgaagctgtgctgggcccctagcccacaggaccggccatcattcagcgccctgggcccccagctggacatgctgtggagcggaagccgggggtgtgagactcatgccttcactgctcacccagagggcaaacaccactccctgtccttttcatagctcctgcccgcagacctctggattaggtctctgttgactggctgtgtgaccttaggcccggagctgcccctctctgggcctcagaggccttatgagggtcctctacttcaggaacacccccatgacattgcatttgggggggctcccgtggcctgtagaatagcctgtggcctttgcaatttgttaaggttcaagacagatgggcatatgtgtcagtggggctctctgagtcctggcccaaagaagcaaggaaccaaatttaagactctcgcatcttcccaaccccttaagccctggccccctgagtttccttttctgtctctctctttttattttttttatttttatttttatttttgagacagagcctcgctctgttacccagggtggagtgcagtggtgcgatctcggctcagtgcaacctctgcttcccaggttcaagcgattctcctgcctcagcctcccgagtagctgggattacaggtgtgcaccaccacacccggctaattttttttatttttaatagagatgaggtttcaccatgatggccaggctgatctcgaactcctaacctcaagtgatcctcccacctcagcctcccaaagtgttggaataataggcatgagccactgcacccaggcttttttttttttaaatttattattattatttttaagagacaggatcttgctacgttgcccaggctggtcttgaactcctgggctacagtgatcctcctgccttatcctcctaaatagctgggactacagcacctagttttgagtttcctgtcttatttccaatggggacattcatgtagctttttttttttttttttttttgagacggagtctcgctctgtcgcccaggctggagtacagtggcgcaatctaggctcactgcaagctccgcctcctgggttcacaccattctctcgcctcagcctcccaagtagctgggactacaggcgcccgccaccacacccggctaattttttgtatttttagtagagacggggtttcaccttgttagccaggatggtttccatctcctgacctcgtgatctgcccgtctcggcctcccaaagtgctgggattacaggcatgagccactgcgcccggccctcatgtagctttaaatgtatgatctgacttctgctccccgatctctgtttctctggaggaagccaaggacaagagcagttgctgtggctgggactctgccttttaggggagcccgtgtatctctttgggatcctgaaagggggcaggaaaggctggggtcccagtccaccctaatggtatctgagtgtcctagggcttcagttttcccacctgtccaatgggaccctttctgtcctcaccctacaaggggcacaaagggatgacaccaaacctggcaggaacttttcacgcaatcaagggaaggaaaggcattcctggcagagggaacagcatgccaagcgtgagaaggctcagagtaaggaggttaagagcccaagtattggagcctacagttttgccccttccatgcagtgtgacagtgggcaagttcctttccctctctgggtctcagttctgtcccctgcaaaatggtcagagcttaccccttggctgtgcagggtcaactttctgactggtgagagggattctcatgcaggttaagcttctgctgctcctcctcacctgcaaagcttttctgccacttttgcctccttggaaaactcttatccatctctcaaaactccagctaccacatccttgcagccttccctcatatacccccactactactgtagccctgtccttccctccagccccactctggccctggggctggggaagtgtctgtgtccagctgtctcccctgacctcagggttccttgggggctgggctgaggcctcagtacagagggggctctggaaatgtttgttgactgaataaaggaattcagtggaaaaaaaaaaaaaaaaa

SEQ ID NO: 14 - DNA, 4064 bp, Homo sapiens
ccctctgaccaggactgaggggctttttctctctgtgccccaggcaagttgcactcattatggaattccggcggcccgctaggcaagttgcactcatggcacctccaagtgaagagacgcccctgatccctcagcgttcatgcagcctcttgtccacggaggctggtgccctgcatgtgctgctgcccgctcgggccccggggcccccccagcgcctatctttctcctttggggaccacttggctgaggacctgtgcgtgcaggctgccaaggccagcggcatcctgcctgtgtaccactccctctttgctctggccacggaggacctgtcctgctggttccccccgagccacatcttctccgtggaggatgccagcacccaagtcctgctgtacaggattcgcttttacttccccaattggtttgggctggagaagtgccaccgcttcgggctacgcaaggatttggccagtgctatccttgacctgccagtcctggagcacctctttgcccagcaccgcagtgacctggtgagtgggcgcctccccgtgggcctcagtctcaaggagcagggtgagtgtctcagcctggccgtgttggacctggcccggatggcgcgagagcaggcccagcggccgggagagctgctgaagactgtcagctacaaggcctgcctacccccaagcctgcgcgacctgatccagggcctgagcttcgtgacgcggagggctattcggaggacggtgcgcagagccctgccgcgcgtggccgcctgccaggcagaccggcactcgctcatggccaagtacatcatggacctggagcggctggatccagccggggccgccgagaccttccacgtgggcctccctggggcccttggtggccacgacgggctggggctgctccgcgtggctggtgacggcggcatcgcctggacccagggagaacaggaggtcctccagcccttctgcgactttccagaaatcgtagacattagcatcaagcaggccccgcgcgttggcccggccggagagcaccgcctggtcactgttaccaggacagacaaccagattttagaggccgagttcccagggctgcccgaggctctgtcgttcgtggcgctcgtggacggctacttccggctgaccacggactcccagcacttcttctgcaaggaggtggcaccgccgaggctgctggaggaagtggccgagcagtgccacggccccatcactctggactttgccatcaacaagctcaagactgggggctcacgtcctggctcctatgttctccgccgcagcccccaggactttgacagcttcctcctcactgtctgtgtccagaacccccttggtcctgattataagggctgcctcatccggcgcagccccacaggaaccttccttctggttggcctcagccgaccccacagcagtcttcgagagctcctggcaacctgctgggatggggggctgcacgtagatggggtggcagtgaccctcacttcctgctgtatccccagacccaaagaaaagtccaacctgatcgtggtccagagaggtcacagcccacccacatcatccttggttcagccccaatcccaataccagctgagtcagatgacatttcacaagatccctgctgacagcctggagtggcatgagaacctgggccatgggtccttcaccaagatttaccggggctgtcgccatgaggtggtggatggggaggcccgaaagacagaggtgctgctgaaggtcatggatgccaagcacaagaactgcatggagtcattcctggaagcagcgagcttgatgagccaagtgtcgtaccggcatctcgtgctgctccacggcgtgtgcatggctggagacagcaccatggtgcaggaatttgtacacctgggggccatagacatgtatctgcgaaaacgtggccacctggtgccagccagctggaagctgcaggtggtcaaacagctggcctacgccctcaactatctggaggacaaaggcctgccccatggcaatgtctctgcccggaaggtgctcctggctcgggagggggctgatgggagcccgcccttcatcaagctgagtgaccctggggtcagccccgctgtgttaagcctggagatgctcaccgacaggatcccctgggtggcccccgagtgtctccgggaggcgcagacacttagcttggaagctgacaagtggggcttcggcgccacggtctgggaagtgtttagtggcgtcaccatgcccatcagtgccctggatcctgctaagaaactccaattttatgaggaccggcagcagctgccggcccccaagtggacagagctggccctgctgattcaacagtgcatggcctatgagccggtccagaggccctccttccgagccgtcattcgtgacctcaatagcctcatctcttcagactatgagctcctctcagaccccacacctggtgccctggcacctcgtgatgggctgtggaatggtgcccagctctatgcctgccaagaccccacgatcttcgaggagagacacctcaagtacatctcacagctgggcaagggcaactttggcagcgtggagctgtgccgctatgacccgctagcccacaatacaggtgccctggtggccgtgaaacagctgcagcacagcgggccagaccagcagagggactttcagcgggagattcagatcctcaaagcactgcacagtgatttcattgtcaagtatcgtggtgtcagctatggcccgggccggccagagctgcggctggtcatggagtacctgcccagcggctgcttgcgcgacttcctgcagcggcaccgcgcgcgcctcgatgccagccgcctccttctctattcctcgcagatctgcaagggcatggagtacctgggctcccgccgctgcgtgcaccgcgacctggccgcccgaaacatcctcgtggagagcgaggcacacgtcaagatcgctgacttcggcctagctaagctgctgccgcttgacaaagactactacgtggtccgcgagccaggccagagccccattttctggtatgcccccgaatccctctcggacaacatcttctctcgccagtcagacgtctggagcttcggggtcgtcctgtacgagctcttcacctactgcgacaaaagctgcagcccctcggccgagttcctgcggatgatgggatgtgagcgggatgtccccgccctctgccgcctcttggaactgctggaggagggccagaggctgccggcgcctcctgcctgccctgctgaggttcacgagctcatgaagctgtgctgggcccctagcccacaggaccggccatcattcagcgccctgggcccccagctggacatgctgtggagcggaagccgggggtgtgagactcatgccttcactgctcacccagagggcaaacaccactccctgtccttttcatagctcctgcccgcagacctctggattaggtctctgttgactggctgtgtgaccttaggcccggagctgcccctctctgggcctcagaggccttatgagggtcctctacttcaggaacacccccatgacattgcatttgggggggctcccgtggcctgtagaatagcctgtggcctttgcaatttgttaaggttcaagacagatgggcatatgtgtcagtggggctctctgagtcctggcccaaagaagcaaggaaccaaatttaagactctcgcatcttcccaaccccttaagccctggccccctgagtttccttttctcgtctctctctttttattttttttatttttatttttatttttgagacagagcctcgctcgttacccagggtggagtgcagtggtagcgatctcggctcacagtgcaacctctgcttcccaggttcaagcgattctcctgcctcagcctcccgagtagctgggattacaggtgtgcaccaccacacccggctaattttttttatttttaatagagatgaggtttcaccatgatggccaggctgatctcgaactcctaacctcaagtgatcctcccacc

SEQ ID NO: 15 - DNA, 4262 bp, Homo sapiens
aagcagtagctacccgcgggagcggggaggggtccgggttcgagcttgtgttcccccggaagggtgagtctggacgcgggcgcggaaggagcgcggccggaggtcctcaggaagaagccgcggggactggctgcgcttgacaggctgcacttggatgggagcacctggtgcctcgggactgctccgatgcccgggtctgtgctgaatgtgtaatatgcggaactatattgaaacattacaaccatcttttgatggcaacaccctgaggacctcccttttccagatggggaaactgaggcccagaattgctaagtggcttgcttgagttgacacagggagctccaggactcaccctcagctgagccacctgccgggagcatgcctctgcgccactgggggatggccaggggcagtaagcccgttggggatggagcccagcccatggctgccatgggaggcctgaaggtgcttctgcactgggctggtccaggcggcggggagccctgggtcactttcagtgagtcatcgctgacagctgaggaagtctgcatccacattgcacataaagttggtatcactcctccttgcttcaatctctttgccctcttcgatgctcaggcccaagtctggttgcccccaaaccacatcctagagatccccagagatgcaagcctgatgctatatttccgcataaggttttatttccggaactggcatggcatgaatcctcgggaaccggctgtgtaccgttgtgggcccccaggaaccgaggcatcctcagatcagacagcacaggggatgcaactcctggacccagcctcatttgagtacctctttgagcagggcaagcatgagtttgtgaatgacgtggcatcactgtgggagctgtcgaccgaggaggagatccaccactttaagaatgagagcctgggcatggcctttctgcacctctgtcacctcgctctccgccatggcatccccctggaggaggtggccaagaagaccagcttcaaggactgcatcccgcgctccttccgccggcatatccggcagcacagcgccctgacccggctgcgccttcggaacgtcttccgcaggttcctgcgggacttccagccgggccgactctcccagcagatggtcatggtcaaatacctagccacactcgagcggctggcaccccgcttcggcacagagcgtgtgcccgtgtgccacctgaggctgctggcccaggccgagggggagccctgctacatccgggacagtggggtggcccctacagaccctggccctgagtctgctgctgggcccccaacccacgaggtgctggtgacaggcactggtggcatccagtggtggccagtagaggaggaggtgaacaaggaggagggttctagtggcagcagtggcaggaacccccaagccagcctgtttgggaagaaggccaaggctcacaaggcagtcggccagccggcagacaggccgcgggagccactgtgggcctacttctgtgacttccgggacatcacccacgtggtgctgaaagagcactgtgtcagcatccaccggcaggacaacaagtgcctggagctgagcttgccttcccgggctgcggcgctgtccttcgtgtcgctggtggacggctatttccgcctgacggccgactccagccactacctgtgccacgaggtggctcccccacggctggtgatgagcatccgggatgggatccacggacccctgctggagccatttgtgcaggccaagctgcggcccgaggacggcctgtacctcattcactggagcaccagccacccctaccgcctgatcctcacagtggcccagcgtagccaggcaccagacggcatgcagagcttgcggctccgaaagttccccattgagcagcaggacggggccttcgtgctggagggctggggccggtccttccccagcgttcgggaacttggggctgccttgcagggctgcttgctgagggccggggatgactgcttctctctgcgtcgctgttgcctgccccaaccaggagaaacctccaatctcatcatcatgcggggggctcgggccagccccaggacactcaacctcagccagctcagcttccaccgggttgaccagaaggagatcacccagctgtcccacttgggccagggcacaaggaccaacgtgtatgagggccgcctgcgagtggagggcagcggggaccctgaggagggcaagatggatgacgaggaccccctcgtgcctggcagggaccgtgggcaggagctacgagtggtgctcaaagtgctggaccctagtcaccatgacatcgccctggccttctacgagacagccagcctcatgagccaggtctcccacacgcacctggccttcgtgcatggcgtctgtgtgcgcggccctgaaaatatcatggtgacagagtacgtggagcacggacccctggatgtgtggctgcggagggagcggggccatgtgcccatggcttggaagatggtggtggcccagcagctggccagcgccctcagctacctggagaacaagaacctggttcatggtaatgtgtgtggccggaacatcctgctggcccggctggggttggcagagggcaccagccccttcatcaagctgagtgatcctggcgtgggcctgggcgccctctccagggaggagcgggtggagaggatcccctggctggcccccgaatgcctaccaggtggggccaacagcctaagcaccgccatggacaagtgggggtttggcgccaccctcctggagatctgctttgacggagaggcccctctgcagagccgcagtccctccgagaaggagcatttctaccagaggcagcaccggctgcccgagccctcctgcccacagctggccacactcaccagccagtgtctgacctatgagccaacccagaggccatcattccgcaccatcctgcgtgacctcacccggctgcagccccacaatcttgctgacgtcttgactgtgaacccggactcaccggcgtcggaccctacggttttccacaagcgctatttgaaaaagatccgagatctgggcgagggtcacttcggcaaggtcagcttgtactgctacgatccgaccaacgacggcactggcgagatggtggcggtgaaagccctcaaggcagactgcggcccccagcaccgctcgggctggaagcaggagattgacattctgcgcacgctctaccacgagcacatcatcaagtacaagggctgctgcgaggaccaaggcgagaagtcgctgcagctggtcatggagtacgtgcccctgggcagcctccgagactacctgccccggcacagcatcgggctggcccagctgctgctcttcgcccagcagatctgcgagggcatggcctatctgcacgcgcagcactacatccaccgagacctagccgcgcgcaacgtgctgctggacaacgacaggctggtcaagatcggggactttggcctagccaaggccgtgcccgaaggccacgagtactaccgcgtgcgcgaggatggggacagccccgtgttctggtatgccccagagtgcctgaaggagtataagttctactatgcgtcagatgtctggtccttcggggtgaccctgtatgagctgctgacgcactgtgactccagccagagcccccccacgaaattccttgagctcataggcattgctcagggtcagatgacagttctgagactcactgagttgctggaacgaggggagaggctgccacggcccgacaaatgtccctgtgaggtctatcatctcatgaagaactgctgggagacagaggcgtcctttcgcccaaccttcgagaacctcatacccattctgaagacagtccatgagaagtaccaaggccaggccccttcagtgttcagcgtgtgctgaggcacaatggcagccctgcctgggaggactggaccaggcagtggctgcagagggagcctcctgctccctgctccaggatgaaaccaagagggggatgtcagcctcacccacaccgtgtgccttactcctgtctagagaccccacctctgtgaacttatttttctttcttggccgtgagcctaaccatgatcttgagggacccaacatttgtaggggcactaatccagcccttaaatcccccagcttccaaacttgaggcccaccatctccaccatctggtaataaactcatgttttctctgctggaaaaaaaaaaaaaaa